European Patent Application EP 4 169 528 A1, published April 26, 2023. Title: ANTIGENIC PEPTIDES FOR PREVENTION AND TREATMENT OF CANCER. Applicant: ENTEROME S.A. The sequence listing filed with the application follows.

SEQUENCE LISTING (899 sequences)

SEQ ID NO: 1 - protein, 9 aa, synthetic construct
  REGION 1..9: note = peptide
VLFLLFFPV

SEQ ID NO: 2 - protein, 9 aa, synthetic construct
  REGION 1..9: note = peptide
SMSLGFLSV

SEQ ID NO: 3 - protein, 9 aa, synthetic construct
  REGION 1..9: note = peptide
FLSLGFLAV

SEQ ID NO: 4 - protein, 9 aa, synthetic construct
  REGION 1..9: note = peptide
LLLGFLFLI

SEQ ID NO: 5 - protein, 9 aa, synthetic construct
  REGION 1..9: note = peptide
YLSNDSYRV

SEQ ID NO: 6 - protein, 9 aa, synthetic construct
  REGION 1..9: note = peptide
GLIDSGAFL

SEQ ID NO: 7 - protein, 9 aa, synthetic construct
  REGION 1..9: note = peptide
LLIDSGALV

SEQ ID NO: 8 - protein, 9 aa, synthetic construct
  REGION 1..9: note = peptide
RLIDSGATV

SEQ ID NO: 9 - protein, 9 aa, synthetic construct
  REGION 1..9: note = peptide
KLFESSAAL

SEQ ID NO: 10 - protein, 9 aa, synthetic construct
  REGION 1..9: note = peptide
TLFESSAFA

SEQ ID NO: 11 - protein, 9 aa, synthetic construct
  REGION 1..9: note = peptide
MLTPLLLGL

SEQ ID NO: 12 - protein, 9 aa, synthetic construct
  REGION 1..9: note = peptide
YLTPLLLIL

SEQ ID NO: 13 - protein, 9 aa, synthetic construct
  REGION 1..9: note = peptide
IMTPLLLPV

SEQ ID NO: 14 - protein, 9 aa, synthetic construct
  REGION 1..9: note = peptide
FMTPLLLCL

SEQ ID NO: 15 - protein, 9 aa, synthetic construct
  REGION 1..9: note = peptide
FLTPLLLWL

SEQ ID NO: 16 - protein, 9 aa, synthetic construct
  REGION 1..9: note = peptide
WMAVILTAL

SEQ ID NO: 17 - protein, 9 aa, synthetic construct
  REGION 1..9: note = peptide
VLAVILTAV

SEQ ID NO: 18 - protein, 9 aa, synthetic construct
  REGION 1..9: note = peptide
VLAAIAAGV

SEQ ID NO: 19 - protein, 9 aa, synthetic construct
  REGION 1..9: note = peptide
LLAAIAAFL

SEQ ID NO: 20 - protein, 9 aa, synthetic construct
  REGION 1..9: note = peptide
KLAAIAAAV

SEQ ID NO: 21 - protein, 9 aa, synthetic construct
  REGION 1..9: note = peptide
ILAAIAAAV

SEQ ID NO: 22 - protein, 9 aa, synthetic construct
  REGION 1..9: note = peptide
GMAAIAAFL

SEQ ID NO: 23 - protein, 9 aa, synthetic construct
  REGION 1..9: note = peptide
FLAAIAAVL

SEQ ID NO: 24 - protein, 9 aa, synthetic construct
  REGION 1..9: note = peptide
ALAAIAALV

SEQ ID NO: 25 - protein, 9 aa, synthetic construct
  REGION 1..9: note = peptide
ALAAFQAGL

SEQ ID NO: 26 - protein, 9 aa, synthetic construct
  REGION 1..9: note = peptide
SLVNLGFSL

SEQ ID NO: 27 - protein, 9 aa, synthetic construct
  REGION 1..9: note = peptide
GLVNLGFAL

SEQ ID NO: 28 - protein, 9 aa, synthetic construct
  REGION 1..9: note = peptide
QLLDFSSSL

SEQ ID NO: 29 - protein, 9 aa, synthetic construct
  REGION 1..9: note = peptide
ILLDFSSVV

SEQ ID NO: 30 - protein, 9 aa, synthetic construct
  REGION 1..9: note = peptide
YTLGEFLYI

SEQ ID NO: 31 - protein, 9 aa, synthetic construct
  REGION 1..9: note = peptide
GLLGEFLQI

SEQ ID NO: 32 - protein, 9 aa, synthetic construct
  REGION 1..9: note = peptide
FMLGEFLKL

SEQ ID NO: 33 - protein, 9 aa, synthetic construct
  REGION 1..9: note = peptide
VLGDILALL

SEQ ID NO: 34 - protein, 9 aa, synthetic construct
  REGION 1..9: note = peptide
KVGDILALV

SEQ ID NO: 35 - protein, 9 aa, synthetic construct
  REGION 1..9: note = peptide
NLVFGLLPV

SEQ ID NO: 36 - protein, 9 aa, synthetic construct
  REGION 1..9: note = peptide
FLVFGLLGL

SEQ ID NO: 37 - protein, 9 aa, synthetic construct
  REGION 1..9: note = peptide
ALVFGLLRV

SEQ ID NO: 38 - protein, 9 aa, synthetic construct
  REGION 1..9: note = peptide
GVYEGSLTV

SEQ ID NO: 39 - protein, 9 aa, synthetic construct
  REGION 1..9: note = peptide
VLSTAFALV

SEQ ID NO: 40 - protein, 9 aa, synthetic construct
  REGION 1..9: note = peptide
GLSTAFAAV

SEQ ID NO: 41 - protein, 9 aa, synthetic construct
  REGION 1..9: note = peptide
ALSTAFAVV

SEQ ID NO: 42 - protein, 9 aa, synthetic construct
  REGION 1..9: note = peptide
MLLLLLVPV

SEQ ID NO: 43 - protein, 9 aa, synthetic construct
  REGION 1..9: note = peptide
LLLLLLVPV

SEQ ID NO: 44 - protein, 9 aa, synthetic construct
  REGION 1..9: note = peptide
AILLLLVPV

SEQ ID NO: 45 - protein, 9 aa, synthetic construct
  REGION 1..9: note = peptide
YLLLSLLRL

SEQ ID NO: 46 - protein, 9 aa, synthetic construct
  REGION 1..9: note = peptide
FLLLSLLTL

SEQ ID NO: 47 - protein, 9 aa, synthetic construct
  REGION 1..9: note = peptide
ALLLSLLPL

SEQ ID NO: 48 - protein, 9 aa, synthetic construct
  REGION 1..9: note = peptide
RLLLLSLLV

SEQ ID NO: 49 - protein, 9 aa, synthetic construct
  REGION 1..9: note = peptide
KLLLLSLLL

SEQ ID NO: 50 - protein, 9 aa, synthetic construct
  REGION 1..9: note = peptide
FLLLLSLLI

SEQ ID NO: 51 - protein, 9 aa, synthetic construct
  REGION 1..9: note = peptide
RLAKYVALV

SEQ ID NO: 52 - protein, 9 aa, synthetic construct
  REGION 1..9: note = peptide
LIAAAAFTV

SEQ ID NO: 53 - protein, 9 aa, synthetic construct
  REGION 1..9: note = peptide
GMAAAAFCL

SEQ ID NO: 54 - protein, 9 aa, synthetic construct
  REGION 1..9: note = peptide
GLAAAAFCI

SEQ ID NO: 55 - protein, 9 aa, synthetic construct
  REGION 1..9: note = peptide
FLAAAAFCL

SEQ ID NO: 56 - protein, 9 aa, synthetic construct
  REGION 1..9: note = peptide
WLNDRVLQL

SEQ ID NO: 57 - protein, 9 aa, synthetic construct
  REGION 1..9: note = peptide
KLLLTTLLV

SEQ ID NO: 58 - protein, 9 aa, synthetic construct
  REGION 1..9: note = peptide
GMAVVFINV

SEQ ID NO: 59 - protein, 9 aa, synthetic construct
  REGION 1..9: note = peptide
GMAVVFIEV

SEQ ID NO: 60 - protein, 9 aa, synthetic construct
  REGION 1..9: note = peptide
LLLTTLLAV

SEQ ID NO: 61 - protein, 9 aa, synthetic construct
  REGION 1..9: note = peptide
ALLTTLLLV

SEQ ID NO: 62 - protein, 9 aa, synthetic construct
  REGION 1..9: note = peptide
ALLTTLLGL

SEQ ID NO: 63 - protein, 9 aa, synthetic construct
  REGION 1..9: note = peptide
KIIGIILAV

SEQ ID NO: 64 - protein, 9 aa, synthetic construct
  REGION 1..9: note = peptide
YLVAILLLV

SEQ ID NO: 65 - protein, 9 aa, synthetic construct
  REGION 1..9: note = peptide
TLVAILLNV

SEQ ID NO: 66 - protein, 9 aa, synthetic construct
  REGION 1..9: note = peptide
MLVAILLAV

SEQ ID NO: 67 - protein, 9 aa, synthetic construct
  REGION 1..9: note = peptide
LLVAILLSV

SEQ ID NO: 68 - protein, 9 aa, synthetic construct
  REGION 1..9: note = peptide
FLVAILLNL

SEQ ID NO: 69 - protein, 9 aa, synthetic construct
  REGION 1..9: note = peptide
AMVAILLNI

SEQ ID NO: 70 - protein, 9 aa, synthetic construct
  REGION 1..9: note = peptide
ALVAILLAI

SEQ ID NO: 71 - protein, 9 aa, synthetic construct
  REGION 1..9: note = peptide
LLSDVGTLL

SEQ ID NO: 72 - protein, 9 aa, synthetic construct
  REGION 1..9: note = peptide
FLSTYLLPM

SEQ ID NO: 73 - protein, 9 aa, synthetic construct
  REGION 1..9: note = peptide
ALLEEYTGI

SEQ ID NO: 74 - protein, 9 aa, synthetic construct
  REGION 1..9: note = peptide
SLLCIVIGL

SEQ ID NO: 75 - protein, 9 aa, synthetic construct
  REGION 1..9: note = peptide
ILLCIVIGL

SEQ ID NO: 76 - protein, 9 aa, synthetic construct
  REGION 1..9: note = peptide
MLVTVVLTV

SEQ ID NO: 77 - protein, 9 aa, synthetic construct
  REGION 1..9: note = peptide
MLVTVVLLV

SEQ ID NO: 78 - protein, 9 aa, synthetic construct
  REGION 1..9: note = peptide
LLVTVVLPV

SEQ ID NO: 79 - protein, 9 aa, synthetic construct
  REGION 1..9: note = peptide
LLVTVVLAV

SEQ ID NO: 80 - protein, 9 aa, synthetic construct
  REGION 1..9: note = peptide
KLVTVVLAV

SEQ ID NO: 81 - protein, 9 aa, synthetic construct
  REGION 1..9: note = peptide
ILVTVVLGI

SEQ ID NO: 82 - protein, 9 aa, synthetic construct
  REGION 1..9: note = peptide
LMALVLMLV

SEQ ID NO: 83 - protein, 9 aa, synthetic construct
  REGION 1..9: note = peptide
GLTFWNPNV

SEQ ID NO: 84 - protein, 9 aa, synthetic construct
  REGION 1..9: note = peptide
FMLLLSAAA

SEQ ID NO: 85 - protein, 9 aa, synthetic construct
  REGION 1..9: note = peptide
FLLLLSAAL

SEQ ID NO: 86 - protein, 9 aa, synthetic construct
  REGION 1..9: note = peptide
YLLSAALTL

SEQ ID NO: 87 - protein, 9 aa, synthetic construct
  REGION 1..9: note = peptide
YLLSAALTI

SEQ ID NO: 88 - protein, 9 aa, synthetic construct
  REGION 1..9: note = peptide
VLLSAALLL

SEQ ID NO: 89 - protein, 9 aa, synthetic construct
  REGION 1..9: note = peptide
VLLSAALFL

SEQ ID NO: 90 - protein, 9 aa, synthetic construct
  REGION 1..9: note = peptide
SLLSAALTV

SEQ ID NO: 91 - protein, 9 aa, synthetic construct
  REGION 1..9: note = peptide
RLLSAALAL

SEQ ID NO: 92 - protein, 9 aa, synthetic construct
  REGION 1..9: note = peptide
LMLSAALLL

SEQ ID NO: 93 - protein, 9 aa, synthetic construct
  REGION 1..9: note = peptide
LMLSAALCV

SEQ ID NO: 94 - protein, 9 aa, synthetic construct
  REGION 1..9: note = peptide
LMLSAALAV

SEQ ID NO: 95 - protein, 9 aa, synthetic construct
  REGION 1..9: note = peptide
LLLSAALWV

SEQ ID NO: 96 - protein, 9 aa, synthetic construct
  REGION 1..9: note = peptide
LLLSAALTV

SEQ ID NO: 97 - protein, 9 aa, synthetic construct
  REGION 1..9: note = peptide
LLLSAALSV

SEQ ID NO: 98 - protein, 9 aa, synthetic construct
  REGION 1..9: note = peptide
LLLSAALMI

SEQ ID NO: 99 - protein, 9 aa, synthetic construct
  REGION 1..9: note = peptide
LLLSAALLL

SEQ ID NO: 100 - protein, 9 aa, synthetic construct
  REGION 1..9: note = peptide
LLLSAALCV

SEQ ID NO: 101 - protein, 9 aa, synthetic construct
  REGION 1..9: note = peptide
LLLSAALAL

SEQ ID NO: 102 - protein, 9 aa, synthetic construct
  REGION 1..9: note = peptide
KLLSAALSV

SEQ ID NO: 103 - protein, 9 aa, synthetic construct
  REGION 1..9: note = peptide
ILLSAALLL

SEQ ID NO: 104 - protein, 9 aa, synthetic construct
  REGION 1..9: note = peptide
ILLSAALGI

SEQ ID NO: 105 - protein, 9 aa, synthetic construct
  REGION 1..9: note = peptide
FLLSAALVV

SEQ ID NO: 106 - protein, 9 aa, synthetic construct
  REGION 1..9: note = peptide
FLLSAALIL

SEQ ID NO: 107 - protein, 9 aa, synthetic construct
  REGION 1..9: note = peptide
ALLSAALML

SEQ ID NO: 108 - protein, 9 aa, synthetic construct
  REGION 1..9: note = peptide
ALLSAALLV

SEQ ID NO: 109 - protein, 9 aa, synthetic construct
  REGION 1..9: note = peptide
ALLSAALLL

SEQ ID NO: 110 - protein, 9 aa, synthetic construct
  REGION 1..9: note = peptide
YMAGAMVQL

SEQ ID NO: 111 - protein, 9 aa, synthetic construct
  REGION 1..9: note = peptide
RMAGAMVPV

SEQ ID NO: 112 - protein, 9 aa, synthetic construct
  REGION 1..9: note = peptide
RLAGAMVDV

SEQ ID NO: 113 - protein, 9 aa, synthetic construct
  REGION 1..9: note = peptide
MMTGFVVLM

SEQ ID NO: 114 - protein, 9 aa, synthetic construct
  REGION 1..9: note = peptide
YLASSETHV

SEQ ID NO: 115 - protein, 9 aa, synthetic construct
  REGION 1..9: note = peptide
SMLSIGGYV

SEQ ID NO: 116 - protein, 9 aa, synthetic construct
  REGION 1..9: note = peptide
LLIYSFARV

SEQ ID NO: 117 - protein, 9 aa, synthetic construct
  REGION 1..9: note = peptide
KLIHELAEV

SEQ ID NO: 118 - protein, 9 aa, synthetic construct
  REGION 1..9: note = peptide
ILIHELAHI

SEQ ID NO: 119 - protein, 9 aa, synthetic construct
  REGION 1..9: note = peptide
HLWAGVVLV

SEQ ID NO: 120 - protein, 9 aa, synthetic construct
  REGION 1..9: note = peptide
RLWDFTVGV

SEQ ID NO: 121 - protein, 9 aa, synthetic construct
  REGION 1..9: note = peptide
VLASSILYI

SEQ ID NO: 122 - protein, 9 aa, synthetic construct
  REGION 1..9: note = peptide
SLASSILQL

SEQ ID NO: 123 - protein, 9 aa, synthetic construct
  REGION 1..9: note = peptide
ALASSILQL

SEQ ID NO: 124 - protein, 9 aa, synthetic construct
  REGION 1..9: note = peptide
FLAVSLAPL

SEQ ID NO: 125 - protein, 9 aa, synthetic construct
  REGION 1..9: note = peptide
ILVGLFVPV

SEQ ID NO: 126 - protein, 9 aa, synthetic construct
  REGION 1..9: note = peptide
ILVGLFVAV

SEQ ID NO: 127 - protein, 9 aa, synthetic construct
  REGION 1..9: note = peptide
YLFVLLAGI

SEQ ID NO: 128 - protein, 9 aa, synthetic construct
  REGION 1..9: note = peptide
SLFVLLAAV

SEQ ID NO: 129 - protein, 9 aa, synthetic construct
  REGION 1..9: note = peptide
KLFVLLALV

SEQ ID NO: 130 - protein, 9 aa, synthetic construct
  REGION 1..9: note = peptide
GIYDFFVKV

SEQ ID NO: 131 - protein, 9 aa, synthetic construct
  REGION 1..9: note = peptide
TIMGTLVSV

SEQ ID NO: 132 - protein, 9 aa, synthetic construct
  REGION 1..9: note = peptide
RVMGTLVGI

SEQ ID NO: 133 - protein, 9 aa, synthetic construct
  REGION 1..9: note = peptide
TLAEGLALA

SEQ ID NO: 134 - protein, 9 aa, synthetic construct
  REGION 1..9: note = peptide
FLAAGLGQV

SEQ ID NO: 135 - protein, 9 aa, synthetic construct
  REGION 1..9: note = peptide
VLESILHPV

SEQ ID NO: 136 - protein, 9 aa, synthetic construct
  REGION 1..9: note = peptide
RMESILHEV

SEQ ID NO: 137 - protein, 9 aa, synthetic construct
  REGION 1..9: note = peptide
ALLAALCYV

SEQ ID NO: 138 - protein, 9 aa, synthetic construct
  REGION 1..9: note = peptide
YLLALLAWL

SEQ ID NO: 139 - protein, 9 aa, synthetic construct
  REGION 1..9: note = peptide
VLLALLAEV

SEQ ID NO: 140 - protein, 9 aa, synthetic construct
  REGION 1..9: note = peptide
SLLALLAFV

SEQ ID NO: 141 - protein, 9 aa, synthetic construct
  REGION 1..9: note = peptide
RLLALLASV

SEQ ID NO: 142 - protein, 9 aa, synthetic construct
  REGION 1..9: note = peptide
RLLALLAAV

SEQ ID NO: 143 - protein, 9 aa, synthetic construct
  REGION 1..9: note = peptide
LLLALLAPV

SEQ ID NO: 144 - protein, 9 aa, synthetic construct
  REGION 1..9: note = peptide
ALLALLASV

SEQ ID NO: 145 - protein, 9 aa, synthetic construct
  REGION 1..9: note = peptide
ILDEAYVRV

SEQ ID NO: 146 - protein, 9 aa, synthetic construct
  REGION 1..9: note = peptide
ALLLLVVGV

SEQ ID NO: 147 - protein, 9 aa, synthetic construct
  REGION 1..9: note = peptide
GLGALLLLV

SEQ ID NO: 148 - protein, 9 aa, synthetic construct
  REGION 1..9: note = peptide
YMQEILHRL

SEQ ID NO: 149 - protein, 9 aa, synthetic construct
  REGION 1..9: note = peptide
TLAVVSLAV

SEQ ID NO: 150 - protein, 9 aa, synthetic construct
  REGION 1..9: note = peptide
LLAVVSLFV

SEQ ID NO: 151 - protein, 9 aa, synthetic construct
  REGION 1..9: note = peptide
YLVGILLVL

SEQ ID NO: 152 - protein, 9 aa, synthetic construct
  REGION 1..9: note = peptide
KVVGILLPI

SEQ ID NO: 153 - protein, 9 aa, synthetic construct
  REGION 1..9: note = peptide
ILVGILLVV

SEQ ID NO: 154 - protein, 9 aa, synthetic construct
  REGION 1..9: note = peptide
FVVGILLQV

SEQ ID NO: 155 - protein, 9 aa, synthetic construct
  REGION 1..9: note = peptide
ILDEAYVRV

SEQ ID NO: 156 - protein, 9 aa, synthetic construct
  REGION 1..9: note = peptide
LLALLPPEV

SEQ ID NO: 157 - protein, 9 aa, synthetic construct
  REGION 1..9: note = peptide
LLALLPPEL

SEQ ID NO: 158 - protein, 9 aa, synthetic construct
  REGION 1..9: note = peptide
AMALLPPEV

SEQ ID NO: 159 - protein, 9 aa, synthetic construct
  REGION 1..9: note = peptide
ALALLPPPV

SEQ ID NO: 160 - protein, 9 aa, synthetic construct
  REGION 1..9: note = peptide
ILISAVVGL

SEQ ID NO: 161 - protein, 9 aa, synthetic construct
  REGION 1..9: note = peptide
IVLGVVFGV

SEQ ID NO: 162 - protein, 9 aa, synthetic construct
  REGION 1..9: note = peptide
IILGVVFGL

SEQ ID NO: 163 - protein, 9 aa, synthetic construct
  REGION 1..9: note = peptide
YLLELLSAL

SEQ ID NO: 164 - protein, 9 aa, synthetic construct
  REGION 1..9: note = peptide
IMWQFLLEL

SEQ ID NO: 165 - protein, 9 aa, synthetic construct
  REGION 1..9: note = peptide
YLLDAEPQL

SEQ ID NO: 166 - protein, 9 aa, synthetic construct
  REGION 1..9: note = peptide
KLTDTLIPL

SEQ ID NO: 167 - protein, 9 aa, synthetic construct
  REGION 1..9: note = peptide
KLTDTLIEL

SEQ ID NO: 168 - protein, 9 aa, synthetic construct
  REGION 1..9: note = peptide
YLLFAPNAV

SEQ ID NO: 169 - protein, 9 aa, synthetic construct
  REGION 1..9: note = peptide
FLLFAPNSA

SEQ ID NO: 170 - protein, 9 aa, synthetic construct
  REGION 1..9: note = peptide
YLDAEPPAV

SEQ ID NO: 171 - protein, 9 aa, synthetic construct
  REGION 1..9: note = peptide
TLNSGVYLI

SEQ ID NO: 172 - protein, 9 aa, synthetic construct
  REGION 1..9: note = peptide
KMNSGVYVI

SEQ ID NO: 173 - protein, 9 aa, synthetic construct
  REGION 1..9: note = peptide
LLIGLVWSL

SEQ ID NO: 174 - protein, 9 aa, synthetic construct
  REGION 1..9: note = peptide
YLYDLLLTV

SEQ ID NO: 175 - protein, 9 aa, synthetic construct
  REGION 1..9: note = peptide
VLYDLLLEV

SEQ ID NO: 176 - protein, 9 aa, synthetic construct
  REGION 1..9: note = peptide
TLYDLLLSL

SEQ ID NO: 177 - protein, 9 aa, synthetic construct
  REGION 1..9: note = peptide
QLYDLLLVA

SEQ ID NO: 178 - protein, 9 aa, synthetic construct
  REGION 1..9: note = peptide
QLYDLLLSL

SEQ ID NO: 179 - protein, 9 aa, synthetic construct
  REGION 1..9: note = peptide
GLYDLLLRI

SEQ ID NO: 180 - protein, 9 aa, synthetic construct
  REGION 1..9: note = peptide
AVYDLLLEV

SEQ ID NO: 181 - protein, 9 aa, synthetic construct
  REGION 1..9: note = peptide
ALYDLLLEV

SEQ ID NO: 182 - protein, 9 aa, synthetic construct
  REGION 1..9: note = peptide
VLLLILSGV

SEQ ID NO: 183 - protein, 9 aa, synthetic construct
  REGION 1..9: note = peptide
VLLLILSEV

SEQ ID NO: 184 - protein, 9 aa, synthetic construct
  REGION 1..9: note = peptide
SLLLILSFV

SEQ ID NO: 185 - protein, 9 aa, synthetic construct
  REGION 1..9: note = peptide
MLLLILSYL

SEQ ID NO: 186 - protein, 9 aa, synthetic construct
  REGION 1..9: note = peptide
ILLLILSGI

SEQ ID NO: 187 - protein, 9 aa, synthetic construct
  REGION 1..9: note = peptide
FLLLILSLL

SEQ ID NO: 188 - protein, 9 aa, synthetic construct
  REGION 1..9: note = peptide
FLLLILSFL

SEQ ID NO: 189 - protein, 9 aa, synthetic construct
  REGION 1..9: note = peptide
SLAQLLLAI

SEQ ID NO: 190 - protein, 9 aa, synthetic construct
  REGION 1..9: note = peptide
MLAQLLLTV

SEQ ID NO: 191 - protein, 9 aa, synthetic construct
  REGION 1..9: note = peptide
KLIHLMAAV

SEQ ID NO: 192 - protein, 9 aa, synthetic construct
  REGION 1..9: note = peptide
FLDKITDLV

SEQ ID NO: 193 - protein, 9 aa, synthetic construct
  REGION 1..9: note = peptide
FLVEDETVI

SEQ ID NO: 194 - protein, 9 aa, synthetic construct
  REGION 1..9: note = peptide
AVFRVLIPV

SEQ ID NO: 195 - protein, 9 aa, synthetic construct
  REGION 1..9: note = peptide
LLSAVLALV

SEQ ID NO: 196 - protein, 9 aa, synthetic construct
  REGION 1..9: note = peptide
LLSAVLALA

SEQ ID NO: 197 - protein, 9 aa, synthetic construct
  REGION 1..9: note = peptide
GISAVLALV

SEQ ID NO: 198 - protein, 9 aa, synthetic construct
  REGION 1..9: note = peptide
NLWAGGFFL

SEQ ID NO: 199 - protein, 9 aa, synthetic construct
  REGION 1..9: note = peptide
YLALLVMLL

SEQ ID NO: 200 - protein, 9 aa, synthetic construct
  REGION 1..9: note = peptide
LLALLVMAV

SEQ ID NO: 201 - protein, 9 aa, synthetic construct
  REGION 1..9: note = peptide
ALALLVMAV

SEQ ID NO: 202 - protein, 9 aa, synthetic construct
  REGION 1..9: note = peptide
TMLSCLLHL

SEQ ID NO: 203 - protein, 9 aa, synthetic construct
  REGION 1..9: note = peptide
MLLSCLLFM

SEQ ID NO: 204 - protein, 9 aa, synthetic construct
  REGION 1..9: note = peptide
LLLSCLLPL

SEQ ID NO: 205 - protein, 9 aa, synthetic construct
  REGION 1..9: note = peptide
LLLSCLLHL

SEQ ID NO: 206 - protein, 9 aa, synthetic construct
  REGION 1..9: note = peptide
ILLSCLLLL

SEQ ID NO: 207 - protein, 9 aa, synthetic construct
  REGION 1..9: note = peptide
FLLSCLLCL

SEQ ID NO: 208 - protein, 9 aa, synthetic construct
  REGION 1..9: note = peptide
ALLSCLLML

SEQ ID NO: 209 - protein, 9 aa, synthetic construct
  REGION 1..9: note = peptide
YVAATLFAL

SEQ ID NO: 210 - protein, 9 aa, synthetic construct
  REGION 1..9: note = peptide
YLYSEIPDI

SEQ ID NO: 211 - protein, 9 aa, synthetic construct
  REGION 1..9: note = peptide
YMASTLVHL

SEQ ID NO: 212 - protein, 9 aa, synthetic construct
  REGION 1..9: note = peptide
QMASTLVYL

SEQ ID NO: 213 - protein, 9 aa, synthetic construct
  REGION 1..9: note = peptide
YQFDKIYSI

SEQ ID NO: 214 - protein, 9 aa, synthetic construct
  REGION 1..9: note = peptide
MMFWLLLVV

SEQ ID NO: 215 - protein, 9 aa, synthetic construct
  REGION 1..9: note = peptide
GMLWEIFGV

SEQ ID NO: 216 - protein, 9 aa, synthetic construct
  REGION 1..9: note = peptide
AMKDGLPEV

SEQ ID NO: 217 - protein, 9 aa, synthetic construct
  REGION 1..9: note = peptide
TLLDISFAA

SEQ ID NO: 218 - protein, 9 aa, synthetic construct
  REGION 1..9: note = peptide
NMLDISFYL

SEQ ID NO: 219 - protein, 9 aa, synthetic construct
  REGION 1..9: note = peptide
ILDISFPLV

SEQ ID NO: 220 - protein, 9 aa, synthetic construct
  REGION 1..9: note = peptide
LMDLSTTEV

SEQ ID NO: 221 - protein, 9 aa, synthetic construct
  REGION 1..9: note = peptide
RLSSYLVEI

SEQ ID NO: 222 - protein, 9 aa, synthetic construct
  REGION 1..9: note = peptide
MVSSYLVEV

SEQ ID NO: 223 - protein, 9 aa, synthetic construct
  REGION 1..9: note = peptide
KVSSYLVEV

SEQ ID NO: 224 - protein, 9 aa, synthetic construct
  REGION 1..9: note = peptide
ILSKILLFA

SEQ ID NO: 225 - protein, 9 aa, synthetic construct
  REGION 1..9: note = peptide
YQLSYSQMV

SEQ ID NO: 226 - protein, 9 aa, synthetic construct
  REGION 1..9: note = peptide
KLLSYSQEL

SEQ ID NO: 227 - protein, 9 aa, synthetic construct
  REGION 1..9: note = peptide
KIAELPFPL

SEQ ID NO: 228 - protein, 9 aa, synthetic construct
  REGION 1..9: note = peptide
YLNESETVL

SEQ ID NO: 229 - protein, 9 aa, synthetic construct
  REGION 1..9: note = peptide
MLVELLKKV

SEQ ID NO: 230 - protein, 9 aa, synthetic construct
  REGION 1..9: note = peptide
KLVELLKLL

SEQ ID NO: 231 - protein, 9 aa, synthetic construct
  REGION 1..9: note = peptide
ALVELLKPL

SEQ ID NO: 232 - protein, 9 aa, synthetic construct
  REGION 1..9: note = peptide
FLASTTPTA

SEQ ID NO: 233 - protein, 9 aa, synthetic construct
  REGION 1..9: note = peptide
SLAREVAAV

SEQ ID NO: 234 - protein, 9 aa, synthetic construct
  REGION 1..9: note = peptide
GMAREVAAV

SEQ ID NO: 235 - protein, 9 aa, synthetic construct
  REGION 1..9: note = peptide
WLLSLAFLL

SEQ ID NO: 236 - protein, 9 aa, synthetic construct
  REGION 1..9: note = peptide
SLLSLAFSA

SEQ ID NO: 237 - protein, 9 aa, synthetic construct
  REGION 1..9: note = peptide
LLLSLAFIL

SEQ ID NO: 238 - protein, 9 aa, synthetic construct
  REGION 1..9: note = peptide
KLNPAQGYV

SEQ ID NO: 239 - protein, 9 aa, synthetic construct
  REGION 1..9: note = peptide
KLWGLATLI

SEQ ID NO: 240 - protein, 9 aa, synthetic construct
  REGION 1..9: note = peptide
VLALGLLAV

SEQ ID NO: 241 - protein, 9 aa, synthetic construct
  REGION 1..9: note = peptide
SLALGLLQV

SEQ ID NO: 242 - protein, 9 aa, synthetic construct
  REGION 1..9: note = peptide
SLALGLLLV

SEQ ID NO: 243 - protein, 9 aa, synthetic construct
  REGION 1..9: note = peptide
MLALGLLEV

SEQ ID NO: 244 - protein, 9 aa, synthetic construct
  REGION 1..9: note = peptide
GLALGLLFV

SEQ ID NO: 245 - protein, 9 aa, synthetic construct
  REGION 1..9: note = peptide
GLALGLLAV

SEQ ID NO: 246 - protein, 9 aa, synthetic construct
  REGION 1..9: note = peptide
FLALGLLFL

SEQ ID NO: 247 - protein, 9 aa, synthetic construct
  REGION 1..9: note = peptide
ALALGLLMV

SEQ ID NO: 248 - protein, 9 aa, synthetic construct
  REGION 1..9: note = peptide
VLLLAGAYV

SEQ ID NO: 249 - protein, 9 aa, synthetic construct
  REGION 1..9: note = peptide
YLYTFLIVL

SEQ ID NO: 250 - protein, 9 aa, synthetic construct
  REGION 1..9: note = peptide
GMYTFLIPM

SEQ ID NO: 251 - protein, 9 aa, synthetic construct
  REGION 1..9: note = peptide
GLYTFLIPM

SEQ ID NO: 252 - protein, 9 aa, synthetic construct
  REGION 1..9: note = peptide
FLISTTFAA

SEQ ID NO: 253 - protein, 9 aa, synthetic construct
  REGION 1..9: note = peptide
ILLDTNYEI

SEQ ID NO: 254 - protein, 9 aa, synthetic construct
  REGION 1..9: note = peptide
FLPFGFILV

SEQ ID NO: 255 - protein, 10 aa, synthetic construct
  REGION 1..10: note = peptide
FLPFGFILPV

SEQ ID NO: 256 - protein, 9 aa, synthetic construct
  REGION 1..9: note = peptide
MLYLLPLSL

SEQ ID NO: 257 - protein, 9 aa, synthetic construct
  REGION 1..9: note = peptide
MLYLLPLAL

SEQ ID NO: 258 - protein, 9 aa, synthetic construct
  REGION 1..9: note = peptide
LLYLLPLFL

SEQ ID NO: 259 - protein, 9 aa, synthetic construct
  REGION 1..9: note = peptide
SMLYNLLAL

SEQ ID NO: 260 - protein, 9 aa, synthetic construct
  REGION 1..9: note = peptide
AMLYNLLAL

SEQ ID NO: 261 - protein, 9 aa, synthetic construct
  REGION 1..9: note = peptide
ALLYNLLAL

SEQ ID NO: 262 - protein, 9 aa, synthetic construct
  REGION 1..9: note = peptide
ILFLVLQRV

SEQ ID NO: 263 - protein, 9 aa, synthetic construct
  REGION 1..9: note = peptide
YLVAAVVLL

SEQ ID NO: 264 - protein, 9 aa, synthetic construct
  REGION 1..9: note = peptide
YLAERAGHV

SEQ ID NO: 265 - protein, 9 aa, synthetic construct
  REGION 1..9: note = peptide
ILVPLFFTL

SEQ ID NO: 266 - protein, 9 aa, synthetic construct
  REGION 1..9: note = peptide
GLVPLFFAL

SEQ ID NO: 267 - protein, 9 aa, synthetic construct
  REGION 1..9: note = peptide
FLVPLFFVV

SEQ ID NO: 268 - protein, 9 aa, synthetic construct
  REGION 1..9: note = peptide
FLVPLFFLL

SEQ ID NO: 269 - protein, 9 aa, synthetic construct
  REGION 1..9: note = peptide
ALVPLFFAL

SEQ ID NO: 270 - protein, 9 aa, synthetic construct
  REGION 1..9: note = peptide
YMLPLLAGA

SEQ ID NO: 271 - protein, 9 aa, synthetic construct
  REGION 1..9: note = peptide
YLLPLLALA

SEQ ID NO: 272 - protein, 9 aa, synthetic construct
  REGION 1..9: note = peptide
WLLPLLAVV

SEQ ID NO: 273 - protein, 9 aa, synthetic construct
  REGION 1..9: note = peptide
WLLPLLACL

SEQ ID NO: 274 - protein, 9 aa, synthetic construct
  REGION 1..9: note = peptide
WLLPLLAAL

SEQ ID NO: 275 - protein, 9 aa, synthetic construct
  REGION 1..9: note = peptide
TLLPLLAAV

SEQ ID NO: 276 - protein, 9 aa, synthetic construct
  REGION 1..9: note = peptide
TLLPLLAAA

SEQ ID NO: 277 - protein, 9 aa, synthetic construct
  REGION 1..9: note = peptide
SLLPLLAGV

SEQ ID NO: 278 - protein, 9 aa, synthetic construct
  REGION 1..9: note = peptide
RLLPLLAVL

SEQ ID NO: 279 - protein, 9 aa, synthetic construct
  REGION 1..9: note = peptide
RLLPLLAAI

SEQ ID NO: 280 - protein, 9 aa, synthetic construct
  REGION 1..9: note = peptide
QLLPLLAYV

SEQ ID NO: 281 - protein, 9 aa, synthetic construct
  REGION 1..9: note = peptide
LLLPLLAGL

SEQ ID NO: 282 - protein, 9 aa, synthetic construct
  REGION 1..9: note = peptide
LLLPLLADL

SEQ ID NO: 283 - protein, 9 aa, synthetic construct
  REGION 1..9: note = peptide
LLLPLLAAA

SEQ ID NO: 284 - protein, 9 aa, synthetic construct
  REGION 1..9: note = peptide
HVLPLLATV

SEQ ID NO: 285 - protein, 9 aa, synthetic construct
  REGION 1..9: note = peptide
HLLPLLAEV

SEQ ID NO: 286 - protein, 9 aa, synthetic construct
  REGION 1..9: note = peptide
GLLPLLAKI

SEQ ID NO: 287 - protein, 9 aa, synthetic construct
  REGION 1..9: note = peptide
GILPLLATV

SEQ ID NO: 288 - protein, 9 aa, synthetic construct
  REGION 1..9: note = peptide
YLSDAVEAV

SEQ ID NO: 289 - protein, 9 aa, synthetic construct
  REGION 1..9: note = peptide
ILREAAMPV

SEQ ID NO: 290 - protein, 9 aa, synthetic construct
  REGION 1..9: note = peptide
FLIPAPESL

SEQ ID NO: 291 - protein, 9 aa, synthetic construct
  REGION 1..9: note = peptide
FLLHGLNLM

SEQ ID NO: 292 - protein, 9 aa, synthetic construct
  REGION 1..9: note = peptide
YMSSLPQGL

SEQ ID NO: 293 - protein, 9 aa, synthetic construct
  REGION 1..9: note = peptide
YMILGVAMI

SEQ ID NO: 294 - protein, 9 aa, synthetic construct
  REGION 1..9: note = peptide
VLILGVAAV

SEQ ID NO: 295 - protein, 9 aa, synthetic construct
  REGION 1..9: note = peptide
SLILGVAAV

SEQ ID NO: 296 - protein, 9 aa, synthetic construct
  REGION 1..9: note = peptide
ILILGVAGI

SEQ ID NO: 297 - protein, 9 aa, synthetic construct
  REGION 1..9: note = peptide
LLDCIIAFL

SEQ ID NO: 298 - protein, 9 aa, synthetic construct
  REGION 1..9: note = peptide
LILGIFISV

SEQ ID NO: 299 - protein, 9 aa, synthetic construct
  REGION 1..9: note = peptide
YLAVLGISL

SEQ ID NO: 300 - protein, 9 aa, synthetic construct
  REGION 1..9: note = peptide
VLAAIVIGV

SEQ ID NO: 301 - protein, 9 aa, synthetic construct
  REGION 1..9: note = peptide
LLACSLAML

SEQ ID NO: 302 - protein, 9 aa, synthetic construct
  REGION 1..9: note = peptide
FVIGIVALV

SEQ ID NO: 303 - protein, 9 aa, synthetic construct
  REGION 1..9: note = peptide
YVVAVPTPV

SEQ ID NO: 304 - protein, 9 aa, synthetic construct
  REGION 1..9: note = peptide
YIVAVPTPV

SEQ ID NO: 305 - protein, 9 aa, synthetic construct
  REGION 1..9: note = peptide
FIVAVPTPI

SEQ ID NO: 306 - protein, 9 aa, synthetic construct
  REGION 1..9: note = peptide
MLKELSPEL

SEQ ID NO: 307 - protein, 9 aa, synthetic construct
  REGION 1..9: note = peptide
FLKELSPGL

SEQ ID NO: 308 - protein, 9 aa, synthetic construct
  REGION 1..9: note = peptide
FVADLVGHV

SEQ ID NO: 309 - protein, 9 aa, synthetic construct
  REGION 1..9: note = peptide
SLLGTLEEL

SEQ ID NO: 310 - protein, 9 aa, synthetic construct
  REGION 1..9: note = peptide
VMLSDVQSV

SEQ ID NO: 311 - protein, 9 aa, synthetic construct
  REGION 1..9: note = peptide
RLLSDVQGL

SEQ ID NO: 312 - protein, 9 aa, synthetic construct
  REGION 1..9: note = peptide
SLILILSSV

SEQ ID NO: 313 - protein, 9 aa, synthetic construct
  REGION 1..9: note = peptide
KLILILSYL

SEQ ID NO: 314 - protein, 9 aa, synthetic construct
  REGION 1..9: note = peptide
ALDAIFGGV

SEQ ID NO: 315 - protein, 9 aa, synthetic construct
  REGION 1..9: note = peptide
FLITKAEEL

SEQ ID NO: 316 - protein, 9 aa, synthetic construct
  REGION 1..9: note = peptide
SLLEELPAL

SEQ ID NO: 317 - protein, 9 aa, synthetic construct
  REGION 1..9: note = peptide
MTLEELPFL

SEQ ID NO: 318 - protein, 9 aa, synthetic construct
  REGION 1..9: note = peptide
IILEYIALL

SEQ ID NO: 319 - protein, 9 aa, synthetic construct
  REGION 1..9: note = peptide
YMVFGIEGI

SEQ ID NO: 320 - protein, 9 aa, synthetic construct
  REGION 1..9: note = peptide
SLSSSSPLV

SEQ ID NO: 321 - protein, 9 aa, synthetic construct
  REGION 1..9: note = peptide
KLDELAHFL

SEQ ID NO: 322 - protein, 9 aa, synthetic construct
  REGION 1..9: note = peptide
FVLEHVVPL

SEQ ID NO: 323 - protein, 9 aa, synthetic construct
  REGION 1..9: note = peptide
YLLGVLLLL

SEQ ID NO: 324 - protein, 9 aa, synthetic construct
  REGION 1..9: note = peptide
YILGVLLTA

SEQ ID NO: 325 - protein, 9 aa, synthetic construct
  REGION 1..9: note = peptide
MLLGVLLLL

SEQ ID NO: 326 - protein, 9 aa, synthetic construct
  REGION 1..9: note = peptide
MILGVLLFL

SEQ ID NO: 327 - protein, 9 aa, synthetic construct
  REGION 1..9: note = peptide
LMLGVLLLA

SEQ ID NO: 328 - protein, 9 aa, synthetic construct
  REGION 1..9: note = peptide
LLLGVLLLL

SEQ ID NO: 329 - protein, 9 aa, synthetic construct
  REGION 1..9: note = peptide
KLLGVLLLV

SEQ ID NO: 330 - protein, 9 aa, synthetic construct
  REGION 1..9: note = peptide
IILGVLLAV

SEQ ID NO: 331 - protein, 9 aa, synthetic construct
  REGION 1..9: note = peptide
FILGVLLSL

SEQ ID NO: 332 - protein, 9 aa, synthetic construct
  REGION 1..9: note = peptide
ALLGVLLLL

SEQ ID NO: 333 - protein, 9 aa, synthetic construct
  REGION 1..9: note = peptide
ALLGVLLLA

SEQ ID NO: 334 - protein, 9 aa, synthetic construct
  REGION 1..9: note = peptide
AILGVLLLV

SEQ ID NO: 335 - protein, 9 aa, synthetic construct
  REGION 1..9: note = peptide
ILAAGVPEL

SEQ ID NO: 336 - protein, 9 aa, synthetic construct
  REGION 1..9: note = peptide
YVSDILSYV

SEQ ID NO: 337 - protein, 9 aa, synthetic construct
  REGION 1..9: note = peptide
YISDILSYV

SEQ ID NO: 338 - protein, 9 aa, synthetic construct
  REGION 1..9: note = peptide
VISDILSFL

SEQ ID NO: 339 - protein, 9 aa, synthetic construct
  REGION 1..9: note = peptide
SMSDILSRL

SEQ ID NO: 340 - protein, 9 aa, synthetic construct
  REGION 1..9: note = peptide
FVSDILSAA

SEQ ID NO: 341 - protein, 9 aa, synthetic construct
  REGION 1..9: note = peptide
WLLAASVTV

SEQ ID NO: 342 - protein, 9 aa, synthetic construct
  REGION 1..9: note = peptide
ILLAASVLV

SEQ ID NO: 343 - protein, 9 aa, synthetic construct
  REGION 1..9: note = peptide
FLLAASVMM

SEQ ID NO: 344 - protein, 9 aa, synthetic construct
  REGION 1..9: note = peptide
ALLAASVLV

SEQ ID NO: 345 - protein, 9 aa, synthetic construct
  REGION 1..9: note = peptide
LLAASVALL

SEQ ID NO: 346 - protein, 9 aa, synthetic construct
  REGION 1..9: note = peptide
LLAASVAGV

SEQ ID NO: 347 - protein, 9 aa, synthetic construct
  REGION 1..9: note = peptide
ILAASVAAV

SEQ ID NO: 348 - protein, 9 aa, synthetic construct
  REGION 1..9: note = peptide
GLAASVAPV

SEQ ID NO: 349 - protein, 9 aa, synthetic construct
  REGION 1..9: note = peptide
ALLRKVAEV

SEQ ID NO: 350 - protein, 9 aa, synthetic construct
  REGION 1..9: note = peptide
SLPELYAWI

SEQ ID NO: 351 - protein, 9 aa, synthetic construct
  REGION 1..9: note = peptide
ILYGKIKYL

SEQ ID NO: 352 - protein, 9 aa, synthetic construct
  REGION 1..9: note = peptide
MLLGLAAFL

SEQ ID NO: 353 - protein, 9 aa, synthetic construct
  REGION 1..9: note = peptide
GLLGLAAFL

SEQ ID NO: 354 - protein, 9 aa, synthetic construct
  REGION 1..9: note = peptide
ALLGLAAFL

SEQ ID NO: 355 - protein, 9 aa, synthetic construct
  REGION 1..9: note = peptide
YLDEVKSLV

SEQ ID NO: 356 - protein, 9 aa, synthetic construct
  REGION 1..9: note = peptide
YLDEVKSLI

SEQ ID NO: 357 - protein, 9 aa, synthetic construct
  REGION 1..9: note = peptide
YLDEVKSIL

SEQ ID NO: 358 - protein, 9 aa, synthetic construct
  REGION 1..9: note = peptide
LLDEVKSLV

SEQ ID NO: 359 - protein, 9 aa, synthetic construct
  REGION 1..9: note = peptide
FILLSLSPV

SEQ ID NO: 360 - protein, 9 aa, synthetic construct
  REGION 1..9: note = peptide
RLFLFSVLV

SEQ ID NO: 361 - protein, 9 aa, synthetic construct
  REGION 1..9: note = peptide
ALTVYLVYL

SEQ ID NO: 362 - protein, 9 aa, synthetic construct
  REGION 1..9: note = peptide
RLLFVAVPI

SEQ ID NO: 363 - protein, 9 aa, synthetic construct
  REGION 1..9: note = peptide
RLLFVAVGL

SEQ ID NO: 364 - protein, 9 aa, synthetic construct
  REGION 1..9: note = peptide
FLLFVAVSV

SEQ ID NO: 365 - protein, 9 aa, synthetic construct
  REGION 1..9: note = peptide
FISLFLFSV

SEQ ID NO: 366 - protein, 9 aa, synthetic construct
  REGION 1..9: note = peptide
LIAGFVALV

SEQ ID NO: 367 - protein, 9 aa, synthetic construct
  REGION 1..9: note = peptide
YLLVLMASI

SEQ ID NO: 368 - protein, 9 aa, synthetic construct
  REGION 1..9: note = peptide
YLVGILLVL

SEQ ID NO: 369 - protein, 9 aa, synthetic construct
  REGION 1..9: note = peptide
KIVGILLGI

SEQ ID NO: 370 - protein, 9 aa, synthetic construct
  REGION 1..9: note = peptide
KIVGILLAV

SEQ ID NO: 371 - protein, 9 aa, synthetic construct
  REGION 1..9: note = peptide
ILVGILLVV

SEQ ID NO: 372 - protein, 9 aa, synthetic construct
  REGION 1..9: note = peptide
GIVGILLNV

SEQ ID NO: 373 - protein, 9 aa, synthetic construct
  REGION 1..9: note = peptide
GIVGILLAV

SEQ ID NO: 374 - protein, 9 aa, synthetic construct
  REGION 1..9: note = peptide
LLAVVLAFV

SEQ ID NO: 375 - protein, 9 aa, synthetic construct
  REGION 1..9: note = peptide
LLAVVLAAV

SEQ ID NO: 376 - protein, 9 aa, synthetic construct
  REGION 1..9: note = peptide
GVLDGTATV

SEQ ID NO: 377 - protein, 9 aa, synthetic construct
  REGION 1..9: note = peptide
ALADTNSYV

SEQ ID NO: 378 - protein, 9 aa, synthetic construct
  REGION 1..9: note = peptide
ALADTNSYL

SEQ ID NO: 379 - protein, 9 aa, synthetic construct
  REGION 1..9: note = peptide
AMQAAIPML

SEQ ID NO: 380 - protein, 9 aa, synthetic construct
  REGION 1..9: note = peptide
IVLDGLDLV

SEQ ID NO: 381 - protein, 9 aa, synthetic construct
  REGION 1..9: note = peptide
AVLDGLDPV

SEQ ID NO: 382 - protein, 9 aa, synthetic construct
  REGION 1..9: note = peptide
YLLALLPLL

SEQ ID NO: 383 - protein, 9 aa, synthetic construct
  REGION 1..9: note = peptide
YLLALLPIL

SEQ ID NO: 384 - protein, 9 aa, synthetic construct
  REGION 1..9: note = peptide
QLLALLPGV

SEQ ID NO: 385 - protein, 9 aa, synthetic construct
  REGION 1..9: note = peptide
LLLALLPTV

SEQ ID NO: 386 - protein, 9 aa, synthetic construct
  REGION 1..9: note = peptide
FLRELLCQL

SEQ ID NO: 387 - protein, 9 aa, synthetic construct
  REGION 1..9: note = peptide
LLYPVPLGV

SEQ ID NO: 388 - protein, 9 aa, synthetic construct
  REGION 1..9: note = peptide
ALFLLSYTV

SEQ ID NO: 389 - protein, 9 aa, synthetic construct
  REGION 1..9: note = peptide
YVLSLLLTL

SEQ ID NO: 390 - protein, 9 aa, synthetic construct
  REGION 1..9: note = peptide
VLLSLLLIV

SEQ ID NO: 391 - protein, 9 aa, synthetic construct
  REGION 1..9: note = peptide
SLLSLLLIL

SEQ ID NO: 392 - protein, 9 aa, synthetic construct
  REGION 1..9: note = peptide
RLLSLLLVL

SEQ ID NO: 393 - protein, 9 aa, synthetic construct
  REGION 1..9: note = peptide
LVLSLLLLV

SEQ ID NO: 394 - protein, 9 aa, synthetic construct
  REGION 1..9: note = peptide
KLLSLLLVL

SEQ ID NO: 395 - protein, 9 aa, synthetic construct
  REGION 1..9: note = peptide
ILLSLLLVL

SEQ ID NO: 396 - protein, 9 aa, synthetic construct
  REGION 1..9: note = peptide
FTLSLLLTL

SEQ ID NO: 397 - protein, 9 aa, synthetic construct
  REGION 1..9: note = peptide
ALLSLLLIL

SEQ ID NO: 398 - protein, 9 aa, synthetic construct
  REGION 1..9: note = peptide
VLFVLSLFL

SEQ ID NO: 399 - protein, 9 aa, synthetic construct
  REGION 1..9: note = peptide
ILFVLSLQL

SEQ ID NO: 400 - protein, 9 aa, synthetic construct
  REGION 1..9: note = peptide
LLLEKQAEV

SEQ ID NO: 401 - protein, 9 aa, synthetic construct
  REGION 1..9: note = peptide
VLSELKLAV

SEQ ID NO: 402 - protein, 9 aa, synthetic construct
  REGION 1..9: note = peptide
RMIEHVLTV

SEQ ID NO: 403 - protein, 9 aa, synthetic construct
  REGION 1..9: note = peptide
QIFDRLIPI

SEQ ID NO: 404 - protein, 9 aa, synthetic construct
  REGION 1..9: note = peptide
GVFDRLIPI

SEQ ID NO: 405 - protein, 9 aa, synthetic construct
  REGION 1..9: note = peptide
YLKEQFQTL

SEQ ID NO: 406 - protein, 9 aa, synthetic construct
  REGION 1..9: note = peptide
SLLDSAFLL

SEQ ID NO: 407 - protein, 9 aa, synthetic construct
  REGION 1..9: note = peptide
MLSLVFSLI

SEQ ID NO: 408 - protein, 9 aa, synthetic construct
  REGION 1..9: note = peptide
LMSLVFSLV

SEQ ID NO: 409 - protein, 9 aa, synthetic construct
  REGION 1..9: note = peptide
WMQILPYQV

SEQ ID NO: 410 - protein, 9 aa, synthetic construct
  REGION 1..9: note = peptide
MMTGFTFGV

SEQ ID NO: 411 - protein, 9 aa, synthetic construct
  REGION 1..9: note = peptide
MLLLLVNLV

SEQ ID NO: 412 - protein, 9 aa, synthetic construct
  REGION 1..9: note = peptide
VLFGLLTFL

SEQ ID NO: 413 - protein, 9 aa, synthetic construct
  REGION 1..9: note = peptide
QLFGLLTDV

SEQ ID NO: 414 - protein, 9 aa, synthetic construct
  REGION 1..9: note = peptide
FLFGLLTMI

SEQ ID NO: 415 - protein, 9 aa, synthetic construct
  REGION 1..9: note = peptide
FLFGLLTDA

SEQ ID NO: 416 - protein, 9 aa, synthetic construct
  REGION 1..9: note = peptide
TLLLSLFLL

SEQ ID NO: 417 - protein, 9 aa, synthetic construct
  REGION 1..9: note = peptide
FILLSLFML

SEQ ID NO: 418 - protein, 9 aa, synthetic construct
  REGION 1..9: note = peptide
ILLPPPPVV

SEQ ID NO: 419 - protein, 9 aa, synthetic construct
  REGION 1..9: note = peptide
VLLTLIFAL

SEQ ID NO: 420 - protein, 9 aa, synthetic construct
  REGION 1..9: note = peptide
RLLTLIFTL

SEQ ID NO: 421 - protein, 9 aa, synthetic construct
  REGION 1..9: note = peptide
QLLTLIFYL

SEQ ID NO: 422 - protein, 9 aa, synthetic construct
  REGION 1..9: note = peptide
LLLTLIFPI

SEQ ID NO: 423 - protein, 9 aa, synthetic construct
  REGION 1..9: note = peptide
FLLTLIFSL

SEQ ID NO: 424 - protein, 9 aa, synthetic construct
  REGION 1..9: note = peptide
VMVAIYFTL

SEQ ID NO: 425 - protein, 9 aa, synthetic construct
  REGION 1..9: note = peptide
LLGALLPAV

SEQ ID NO: 426 - protein, 9 aa, synthetic construct
  REGION 1..9: note = peptide
ILGALLPLL

SEQ ID NO: 427 - protein, 9 aa, synthetic construct
  REGION 1..9: note = peptide
SVAAFPVTV

SEQ ID NO: 428 - protein, 9 aa, synthetic construct
  REGION 1..9: note = peptide
LLLSLFCLI

SEQ ID NO: 429 - protein, 9 aa, synthetic construct
  REGION 1..9: note = peptide
KLLSLFCTL

SEQ ID NO: 430 - protein, 9 aa, synthetic construct
  REGION 1..9: note = peptide
FLLSLFCIA

SEQ ID NO: 431 - protein, 9 aa, synthetic construct
  REGION 1..9: note = peptide
ILLGVGFGI

SEQ ID NO: 432 - protein, 9 aa, synthetic construct
  REGION 1..9: note = peptide
ALLGVGFGI

SEQ ID NO: 433 - protein, 9 aa, synthetic construct
  REGION 1..9: note = peptide
RLIDEFQSV

SEQ ID NO: 434 - protein, 9 aa, synthetic construct
  REGION 1..9: note = peptide
FLESVITTV

SEQ ID NO: 435 - protein, 9 aa, synthetic construct
  REGION 1..9: note = peptide
GLFGVLIGV

SEQ ID NO: 436 - protein, 9 aa, synthetic construct
  REGION 1..9: note = peptide
AMFGVLISV

SEQ ID NO: 437 - protein, 9 aa, synthetic construct
  REGION 1..9: note = peptide
FIDFLLSEV

SEQ ID NO: 438 - protein, 9 aa, synthetic construct
  REGION 1..9: note = peptide
GLFMVIAGV

SEQ ID NO: 439 - protein, 9 aa, synthetic construct
  REGION 1..9: note = peptide
FLFMVIAFA

SEQ ID NO: 440 - protein, 9 aa, synthetic construct
  REGION 1..9: note = peptide
HLPYLLFLL

SEQ ID NO: 441 - protein, 9 aa, synthetic construct
  REGION 1..9: note = peptide
TLTACLVGV

SEQ ID NO: 442 - protein, 9 aa, synthetic construct
  REGION 1..9: note = peptide
MLSEKMVQL

SEQ ID NO: 443 - protein, 9 aa, synthetic construct
  REGION 1..9: note = peptide
NLFDLSLVA

SEQ ID NO: 444 - protein, 9 aa, synthetic construct
  REGION 1..9: note = peptide
GLFDLSLRV

SEQ ID NO: 445 - protein, 9 aa, synthetic construct
  REGION 1..9: note = peptide
ALFDLSLPI

SEQ ID NO: 446 - protein, 9 aa, synthetic construct
  REGION 1..9: note = peptide
TLPAVMAEV

SEQ ID NO: 447 - protein, 9 aa, synthetic construct
  REGION 1..9: note = peptide
LLAEPQASL

SEQ ID NO: 448 - protein, 9 aa, synthetic construct
  REGION 1..9: note = peptide
ILAEPQALV

SEQ ID NO: 449 - protein, 9 aa, synthetic construct
  REGION 1..9: note = peptide
FIAEPQAAL

SEQ ID NO: 450 - protein, 9 aa, synthetic construct
  REGION 1..9: note = peptide
LLFLLSALL

SEQ ID NO: 451 - protein, 9 aa, synthetic construct
  REGION 1..9: note = peptide
KMLTFLYTA

SEQ ID NO: 452 - protein, 9 aa, synthetic construct
  REGION 1..9: note = peptide
AVLHAIYGV

SEQ ID NO: 453 - protein, 9 aa, synthetic construct
  REGION 1..9: note = peptide
HLFAVLHAV

SEQ ID NO: 454 - protein, 9 aa, synthetic construct
  REGION 1..9: note = peptide
SVIAAIVLV

SEQ ID NO: 455 - protein, 9 aa, synthetic construct
  REGION 1..9: note = peptide
FVIAAIVCV

SEQ ID NO: 456 - protein, 9 aa, synthetic construct
  REGION 1..9: note = peptide
FIIAAIVAV

SEQ ID NO: 457 - protein, 9 aa, synthetic construct
  REGION 1..9: note = peptide
AVIAAIVGV

SEQ ID NO: 458 - protein, 9 aa, synthetic construct
  REGION 1..9: note = peptide
YIAAIIAEA

SEQ ID NO: 459 - protein, 9 aa, synthetic construct
  REGION 1..9: note = peptide
FVAAIIASL

SEQ ID NO: 460 - protein, 9 aa, synthetic construct
  REGION 1..9: note = peptide
FIAAIIAPI

SEQ ID NO: 461 - protein, 9 aa, synthetic construct
  REGION 1..9: note = peptide
GLFKSILFL

SEQ ID NO: 462 - protein, 9 aa, synthetic construct
  REGION 1..9: note = peptide
MLLGTIHGV

SEQ ID NO: 463 - protein, 9 aa, synthetic construct
  REGION 1..9: note = peptide
LLSFFFAML

SEQ ID NO: 464 - protein, 9 aa, synthetic construct
  REGION 1..9: note = peptide
LLSFFFAAL

SEQ ID NO: 465 - protein, 9 aa, synthetic construct
  REGION 1..9: note = peptide
FLSFFFAAM

SEQ ID NO: 466 - protein, 9 aa, synthetic construct
  REGION 1..9: note = peptide
FLAVFLPVL

SEQ ID NO: 467 - protein, 9 aa, synthetic construct
  REGION 1..9: note = peptide
SLLLGTILV

SEQ ID NO: 468 - protein, 9 aa, synthetic construct
  REGION 1..9: note = peptide
ILLLGTILL

SEQ ID NO: 469 - protein, 9 aa, synthetic construct
  REGION 1..9: note = peptide
RLSLIVALV

SEQ ID NO: 470 - protein, 9 aa, synthetic construct
  REGION 1..9: note = peptide
RLSLIVAFV

SEQ ID NO: 471 - protein, 9 aa, synthetic construct
  REGION 1..9: note = peptide
MISPNLFRV

SEQ ID NO: 472 - protein, 9 aa, synthetic construct
  REGION 1..9: note = peptide
LLDHVLIAV

SEQ ID NO: 473 - protein, 9 aa, synthetic construct
  REGION 1..9: note = peptide
RLIDEHLVV

SEQ ID NO: 474 - protein, 9 aa, synthetic construct
  REGION 1..9: note = peptide
TLSEVLEYL

SEQ ID NO: 475 - protein, 9 aa, synthetic construct
  REGION 1..9: note = peptide
FLLRPDTFL

SEQ ID NO: 476 - protein, 9 aa, synthetic construct
  REGION 1..9: note = peptide
LMMTIINQV

SEQ ID NO: 477 - protein, 9 aa, synthetic construct
  REGION 1..9: note = peptide
LLMTIINQV

SEQ ID NO: 478 - protein, 9 aa, synthetic construct
  REGION 1..9: note = peptide
FLMTIINQV

SEQ ID NO: 479 - protein, 9 aa, synthetic construct
  REGION 1..9: note = peptide
RLAGSVAGV

SEQ ID NO: 480 - protein, 9 aa, synthetic construct
  REGION 1..9: note = peptide
KLAGSVAGV

SEQ ID NO: 481 - protein, 9 aa, synthetic construct
  REGION 1..9: note = peptide
LLMMTIITV

SEQ ID NO: 482 - protein, 9 aa, synthetic construct
  REGION 1..9: note = peptide
AMLSSLAGV

SEQ ID NO: 483 - protein, 9 aa, synthetic construct
  REGION 1..9: note = peptide
YVFTMLSAV

SEQ ID NO: 484 - protein, 9 aa, synthetic construct
  REGION 1..9: note = peptide
YLAGVIILI

SEQ ID NO: 485 - protein, 9 aa, synthetic construct
  REGION 1..9: note = peptide
MLAGVIIYI

SEQ ID NO: 486 - protein, 9 aa, synthetic construct
  REGION 1..9: note = peptide
MLAGVIIGI

SEQ ID NO: 487 - protein, 9 aa, synthetic construct
  REGION 1..9: note = peptide
LLAGVIITI

SEQ ID NO: 488 - protein, 9 aa, synthetic construct
  REGION 1..9: note = peptide
LLAGVIIGI

SEQ ID NO: 489 - protein, 9 aa, synthetic construct
  REGION 1..9: note = peptide
GLAGVIITI

SEQ ID NO: 490 - protein, 9 aa, synthetic construct
  REGION 1..9: note = peptide
GLAGVIIAV

SEQ ID NO: 491 - protein, 9 aa, synthetic construct
  REGION 1..9: note = peptide
VMLFGVFMV

SEQ ID NO: 492 - protein, 9 aa, synthetic construct
  REGION 1..9: note = peptide
VLLFGVFLV

SEQ ID NO: 493 - protein, 9 aa, synthetic construct
  REGION 1..9: note = peptide
ILLFGVFMV

SEQ ID NO: 494 - protein, 9 aa, synthetic construct
  REGION 1..9: note = peptide
FILFGVFML

SEQ ID NO: 495 - protein, 9 aa, synthetic construct
  REGION 1..9: note = peptide
VLFGVFLGV

SEQ ID NO: 496 - protein, 9 aa, synthetic construct
  REGION 1..9: note = peptide
GMFGVFLTL

SEQ ID NO: 497 - protein, 9 aa, synthetic construct
  REGION 1..9: note = peptide
FLFGVFLAM

SEQ ID NO: 498 - protein, 9 aa, synthetic construct
  REGION 1..9: note = peptide
VLDTAIIYI

SEQ ID NO: 499 - protein, 9 aa, synthetic construct
  REGION 1..9: note = peptide
KLDTAIIHV

SEQ ID NO: 500 - protein, 9 aa, synthetic construct
  REGION 1..9: note = peptide
LISSFAFLV

SEQ ID NO: 501 - protein, 9 aa, synthetic construct
  REGION 1..9: note = peptide
LISSFAFLL

SEQ ID NO: 502 - protein, 9 aa, synthetic construct
  REGION 1..9: note = peptide
FMLRLIINL

SEQ ID NO: 503 - protein, 9 aa, synthetic construct
  REGION 1..9: note = peptide
ALAIALFPV

SEQ ID NO: 504 - protein, 9 aa, synthetic construct
  REGION 1..9: note = peptide
ALWLHTSFA

SEQ ID NO: 505 - protein, 9 aa, synthetic construct
  REGION 1..9: note = peptide
TMFGYTVFL

SEQ ID NO: 506 - protein, 9 aa, synthetic construct
  REGION 1..9: note = peptide
YLAGIVFTL

SEQ ID NO: 507 - protein, 9 aa, synthetic construct
  REGION 1..9: note = peptide
LMLLFAYYL

SEQ ID NO: 508 - protein, 9 aa, synthetic construct
  REGION 1..9: note = peptide
YLFAYVLIV

SEQ ID NO: 509 - protein, 9 aa, synthetic construct
  REGION 1..9: note = peptide
TLFAYVLGL

SEQ ID NO: 510 - protein, 9 aa, synthetic construct
  REGION 1..9: note = peptide
GLLFAYVEV

SEQ ID NO: 511 - protein, 9 aa, synthetic construct
  REGION 1..9: note = peptide
KILYSLVEV

SEQ ID NO: 512 - protein, 9 aa, synthetic construct
  REGION 1..9: note = peptide
FLLLVNLLV

SEQ ID NO: 513 - protein, 9 aa, synthetic construct
  REGION 1..9: note = peptide
VIADVIALL

SEQ ID NO: 514 - protein, 9 aa, synthetic construct
  REGION 1..9: note = peptide
QIADVIAFL

SEQ ID NO: 515 - protein, 9 aa, synthetic construct
  REGION 1..9: note = peptide
LVADVIASV

SEQ ID NO: 516 - protein, 9 aa, synthetic construct
  REGION 1..9: note = peptide
LIADVIALL

SEQ ID NO: 517 - protein, 9 aa, synthetic construct
  REGION 1..9: note = peptide
LLYSLVFFL

SEQ ID NO: 518 - protein, 9 aa, synthetic construct
  REGION 1..9: note = peptide
FLVKINTNI

SEQ ID NO: 519 - protein, 9 aa, synthetic construct
  REGION 1..9: note = peptide
KLDSLGFTL

SEQ ID NO: 520 - protein, 9 aa, synthetic construct
  REGION 1..9: note = peptide
KLDSLGFSL

SEQ ID NO: 521 - protein, 9 aa, synthetic construct
  REGION 1..9: note = peptide
FLDSLGFSL

SEQ ID NO: 522 - protein, 9 aa, synthetic construct
  REGION 1..9: note = peptide
FMRDEFPDV

SEQ ID NO: 523 - protein, 9 aa, synthetic construct
  REGION 1..9: note = peptide
FLRDEFPEA

SEQ ID NO: 524 - protein, 9 aa, synthetic construct
  REGION 1..9: note = peptide
SMEELLWFV

SEQ ID NO: 525 - protein, 9 aa, synthetic construct
  REGION 1..9: note = peptide
YLLAGLVLL

SEQ ID NO: 526 - protein, 9 aa, synthetic construct
  REGION 1..9: note = peptide
YLLAGLVLI

SEQ ID NO: 527 - protein, 9 aa, synthetic construct
  REGION 1..9: note = peptide
WLVGAVLTL

SEQ ID NO: 528 - protein, 9 aa, synthetic construct
  REGION 1..9: note = peptide
LLVGAVLTV

SEQ ID NO: 529 - protein, 9 aa, synthetic construct
  REGION 1..9: note = peptide
ALVGAVLTV

SEQ ID NO: 530 - protein, 9 aa, synthetic construct
  REGION 1..9: note = peptide
ALVGAVLLV

SEQ ID NO: 531 - protein, 9 aa, synthetic construct
  REGION 1..9: note = peptide
CLSDYVIPV

SEQ ID NO: 532 - protein, 9 aa, synthetic construct
  REGION 1..9: note = peptide
KLAGLVSSV

SEQ ID NO: 533 - protein, 9 aa, synthetic construct
  REGION 1..9: note = peptide
GMSPASFFA

SEQ ID NO: 534 - protein, 9 aa, synthetic construct
  REGION 1..9: note = peptide
ALGAVLTAV

SEQ ID NO: 535 - protein, 9 aa, synthetic construct
  REGION 1..9: note = peptide
YLTALLAEM

SEQ ID NO: 536 - protein, 9 aa, synthetic construct
  REGION 1..9: note = peptide
VLTALLAAV

SEQ ID NO: 537 - protein, 9 aa, synthetic construct
  REGION 1..9: note = peptide
RLTALLAAV

SEQ ID NO: 538 - protein, 9 aa, synthetic construct
  REGION 1..9: note = peptide
GLTALLAPV

SEQ ID NO: 539 - protein, 9 aa, synthetic construct
  REGION 1..9: note = peptide
FLTALLATV

SEQ ID NO: 540 - protein, 9 aa, synthetic construct
  REGION 1..9: note = peptide
TLTESLLYL

SEQ ID NO: 541 - protein, 9 aa, synthetic construct
  REGION 1..9: note = peptide
KLTESLLTI

SEQ ID NO: 542 - protein, 9 aa, synthetic construct
  REGION 1..9: note = peptide
ILTESLLFL

SEQ ID NO: 543 - protein, 9 aa, synthetic construct
  REGION 1..9: note = peptide
RLALLSPYI

SEQ ID NO: 544 - protein, 9 aa, synthetic construct
  REGION 1..9: note = peptide
SILGFIIAA

SEQ ID NO: 545 - protein, 9 aa, synthetic construct
  REGION 1..9: note = peptide
LILGFIIAV

SEQ ID NO: 546 - protein, 9 aa, synthetic construct
  REGION 1..9: note = peptide
FVLGFIITI

SEQ ID NO: 547 - protein, 9 aa, synthetic construct
  REGION 1..9: note = peptide
FILGFIITI

SEQ ID NO: 548 - protein, 9 aa, synthetic construct
  REGION 1..9: note = peptide
SLSGLLSGV

SEQ ID NO: 549 - protein, 9 aa, synthetic construct
  REGION 1..9: note = peptide
FLSGLLSAL

SEQ ID NO: 550 - protein, 9 aa, synthetic construct
  REGION 1..9: note = peptide
ILPLILITV

SEQ ID NO: 551 - protein, 9 aa, synthetic construct
  REGION 1..9: note = peptide
MLGFIIAFL

SEQ ID NO: 552 - protein, 9 aa, synthetic construct
  REGION 1..9: note = peptide
LLGFIIAEV

SEQ ID NO: 553 - protein, 9 aa, synthetic construct
  REGION 1..9: note = peptide
ILGFIIAAV

SEQ ID NO: 554 - protein, 9 aa, synthetic construct
  REGION 1..9: note = peptide
FLGFIIADV

SEQ ID NO: 555 - protein, 9 aa, synthetic construct
  REGION 1..9: note = peptide
MIITVLLLV

SEQ ID NO: 556 - protein, 9 aa, synthetic construct
  REGION 1..9: note = peptide
FIITVLLGL

SEQ ID NO: 557 - protein, 9 aa, synthetic construct
  REGION 1..9: note = peptide
YQIGDSVLL

SEQ ID NO: 558 - protein, 9 aa, synthetic construct
  REGION 1..9: note = peptide
MLSSLIIPL

SEQ ID NO: 559 - protein, 9 aa, synthetic construct
  REGION 1..9: note = peptide
ILIDGAYTV

SEQ ID NO: 560 - protein, 9 aa, synthetic construct
  REGION 1..9: note = peptide
YLLEEGSSV

SEQ ID NO: 561 - protein, 9 aa, synthetic construct
  REGION 1..9: note = peptide
YMFGFTLTM

SEQ ID NO: 562 - protein, 9 aa, synthetic construct
  REGION 1..9: note = peptide
YLFGFTLGM

SEQ ID NO: 563 - protein, 9 aa, synthetic construct
  REGION 1..9: note = peptide
VLFGFTLSI

SEQ ID NO: 564 - protein, 9 aa, synthetic construct
  REGION 1..9: note = peptide
RMFGFTLML

SEQ ID NO: 565 - protein, 9 aa, synthetic construct
  REGION 1..9: note = peptide
LMFGFTLRT

SEQ ID NO: 566 - protein, 9 aa, synthetic construct
  REGION 1..9: note = peptide
YLLFGFTRV

SEQ ID NO: 567 - protein, 9 aa, synthetic construct
  REGION 1..9: note = peptide
VLGPLAALV

SEQ ID NO: 568 - protein, 9 aa, synthetic construct
  REGION 1..9: note = peptide
ILGPLAAWL

SEQ ID NO: 569 - protein, 9 aa, synthetic construct
  REGION 1..9: note = peptide
SLNALLPYV

SEQ ID NO: 570 - protein, 9 aa, synthetic construct
  REGION 1..9: note = peptide
MMIPQVATL

SEQ ID NO: 571 - protein, 9 aa, synthetic construct
  REGION 1..9: note = peptide
MMIPQVATI

SEQ ID NO: 572 - protein, 9 aa, synthetic construct
  REGION 1..9: note = peptide
YLSDIQNAI

SEQ ID NO: 573 - protein, 9 aa, synthetic construct
  REGION 1..9: note = peptide
VMSDIQNRV

SEQ ID NO: 574 - protein, 9 aa, synthetic construct
  REGION 1..9: note = peptide
YQAVVLPGL

SEQ ID NO: 575 - protein, 9 aa, synthetic construct
  REGION 1..9: note = peptide
LLLEQFLSV

SEQ ID NO: 576 - protein, 9 aa, synthetic construct
  REGION 1..9: note = peptide
LLLEQFLAI

SEQ ID NO: 577 - protein, 9 aa, synthetic construct
  REGION 1..9: note = peptide
ALLEQFLTA

SEQ ID NO: 578 - protein, 9 aa, synthetic construct
  REGION 1..9: note = peptide
GVSGYISPV

SEQ ID NO: 579 - protein, 9 aa, synthetic construct
  REGION 1..9: note = peptide
KLTDISSLV

SEQ ID NO: 580 - protein, 9 aa, synthetic construct
  REGION 1..9: note = peptide
YLLSNFYTV

SEQ ID NO: 581 - protein, 9 aa, Homo sapiens
FLFLLFFWL

SEQ ID NO: 582 - protein, 9 aa, Homo sapiens
SLSLGFLFL

SEQ ID NO: 583 - protein, 9 aa, Homo sapiens
LSLGFLFLL

SEQ ID NO: 584 - protein, 9 aa, Homo sapiens
YTSNDSYIV

SEQ ID NO: 585 - protein, 9 aa, Homo sapiens
ILIDSGADI

SEQ ID NO: 586 - protein, 9 aa, Homo sapiens
SLFESSAKI

SEQ ID NO: 587 - protein, 9 aa, Homo sapiens
SLTPLLLSI

SEQ ID NO: 588 - protein, 9 aa, Homo sapiens
MSAVILTAV

SEQ ID NO: 589 - protein, 9 aa, Homo sapiens
ALAAIAAFM

SEQ ID NO: 590 - protein, 9 aa, Homo sapiens
VSAAFQAGV

SEQ ID NO: 591 - protein, 9 aa, Homo sapiens
KLVNLGFQA

SEQ ID NO: 592 - protein, 9 aa, Homo sapiens
ELLDFSSWL

SEQ ID NO: 593 - protein, 9 aa, Homo sapiens
LTLGEFLKL

SEQ ID NO: 594 - protein, 9 aa, Homo sapiens
AAGDILALV

SEQ ID NO: 595 - protein, 9 aa, Homo sapiens
ALVFGLLFA

SEQ ID NO: 596 - protein, 9 aa, Homo sapiens
FQYEGSLTT

SEQ ID NO: 597 - protein, 9 aa, Homo sapiens
HLSTAFARV

SEQ ID NO: 598 - protein, 9 aa, Homo sapiens
LSLLLLVPV

SEQ ID NO: 599 - protein, 9 aa, Homo sapiens
QLLLSLLLL

SEQ ID NO: 600 - protein, 9 aa, Homo sapiens
VQLLLSLLL

SEQ ID NO: 601 - protein, 9 aa, Homo sapiens
NLAKYVAEL

SEQ ID NO: 602 - protein, 9 aa, Homo sapiens
LIAAAAFCL

SEQ ID NO: 603 - protein, 9 aa, Homo sapiens
LLNDRVLRA

SEQ ID NO: 604 - protein, 9 aa, Homo sapiens
GILLTTLLV

SEQ ID NO: 605 - protein, 9 aa, Homo sapiens
ILAVVFIRI

SEQ ID NO: 606 - protein, 9 aa, Homo sapiens
ILLTTLLVI

SEQ ID NO: 607 - protein, 9 aa, Homo sapiens
LVIGIILAV

SEQ ID NO: 608 - protein, 9 aa, Homo sapiens
ALVAILLCI

SEQ ID NO: 609 - protein, 9 aa, Homo sapiens
EMSDVGTFV

SEQ ID NO: 610 - protein, 9 aa, Homo sapiens
EMSTYLLPV

SEQ ID NO: 611 - protein, 9 aa, Homo sapiens
FLLEEYTGS

SEQ ID NO: 612 - protein, 9 aa, Homo sapiens
ILLCIVILL

SEQ ID NO: 613 - protein, 9 aa, Homo sapiens
LLVTVVLFA

SEQ ID NO: 614 - protein, 9 aa, Homo sapiens
AVALVLMLL

SEQ ID NO: 615 - protein, 9 aa, Homo sapiens
LLTFWNPPT

SEQ ID NO: 616 - protein, 9 aa, Homo sapiens
KQLLLSAAL

SEQ ID NO: 617 - protein, 9 aa, Homo sapiens
LLLSAALSA

SEQ ID NO: 618 - protein, 9 aa, Homo sapiens
QLAGAMVWA

SEQ ID NO: 619 - protein, 9 aa, Homo sapiens
SQTGFVVLV

SEQ ID NO: 620 - protein, 9 aa, Homo sapiens
TLASSETGV

SEQ ID NO: 621 - protein, 9 aa, Homo sapiens
ILLSIGGYL

SEQ ID NO: 622 - protein, 9 aa, Homo sapiens
HLIYSFASI

SEQ ID NO: 623 - protein, 9 aa, Homo sapiens
VLIHELAEA

SEQ ID NO: 624 - protein, 9 aa, Homo sapiens
SLWAGVVVL

SEQ ID NO: 625 - protein, 9 aa, Homo sapiens
WLWDFTVTT

SEQ ID NO: 626 - protein, 9 aa, Homo sapiens
LLASSILCA

SEQ ID NO: 627 - protein, 9 aa, Homo sapiens
KLAVSLAET

SEQ ID NO: 628 - protein, 9 aa, Homo sapiens
ALVGLFVLL

SEQ ID NO: 629 - protein, 9 aa, Homo sapiens
GLFVLLAFL

SEQ ID NO: 630 - protein, 9 aa, Homo sapiens
SVYDFFVWL

SEQ ID NO: 631 - protein, 9 aa, Homo sapiens
VVMGTLVAL

SEQ ID NO: 632 - protein, 9 aa, Homo sapiens
GTAEGLALA

SEQ ID NO: 633 - protein, 9 aa, Homo sapiens
GLAAGLGPA

SEQ ID NO: 634 - protein, 9 aa, Homo sapiens
ALESILHRI

SEQ ID NO: 635 - protein, 9 aa, Homo sapiens
ALLAALCPA

SEQ ID NO: 636 - protein, 9 aa, Homo sapiens
ALLALLAAL

SEQ ID NO: 637 - protein, 9 aa, Homo sapiens
ILDEAYVMA

SEQ ID NO: 638 - protein, 9 aa, Homo sapiens
LLLLLVVAL

SEQ ID NO: 639 - protein, 9 aa, Homo sapiens
MVGALLLLL

SEQ ID NO: 640 - protein, 9 aa, Homo sapiens
NLQEILHGA

SEQ ID NO: 641 - protein, 9 aa, Homo sapiens
SLAVVSLNI

SEQ ID NO: 642 - protein, 9 aa, Homo sapiens
AVVGILLVV

SEQ ID NO: 643 - protein, 9 aa, Homo sapiens
ILDEAYVMA

SEQ ID NO: 644 - protein, 9 aa, Homo sapiens
LLALLPPGA

SEQ ID NO: 645 - protein, 9 aa, Homo sapiens
SIISAVVGI

SEQ ID NO: 646 - protein, 9 aa, Homo sapiens
VVLGVVFGI

SEQ ID NO: 647 - protein, 9 aa, Homo sapiens
FLLELLSDS

SEQ ID NO: 648 - protein, 9 aa, Homo sapiens
ALLDAEPPI

SEQ ID NO: 649 - protein, 9 aa, Homo sapiens
KITDTLIHL

SEQ ID NO: 650 - protein, 9 aa, Homo sapiens
KLLFAPNLL

SEQ ID NO: 651 - protein, 9 aa, Homo sapiens
LLDAEPPIL

SEQ ID NO: 652 - protein, 9 aa, Homo sapiens
LLNSGVYTF

SEQ ID NO: 653 - protein, 9 aa, Homo sapiens
LMIGLVWRS

SEQ ID NO: 654 - protein, 9 aa, Homo sapiens
PLYDLLLEM

SEQ ID NO: 655 - protein, 9 aa, Homo sapiens
QLLLILSHI

SEQ ID NO: 656 - protein, 9 aa, Homo sapiens
RLAQLLLIL

SEQ ID NO: 657 - protein, 9 aa, Homo sapiens
TLIHLMAKA

SEQ ID NO: 658 - protein, 9 aa, Homo sapiens
VLDKITDTL

SEQ ID NO: 659 - protein, 9 aa, Homo sapiens
FMVEDETVL

SEQ ID NO: 660 - protein, 9 aa, Homo sapiens
SMFRVLIGT

SEQ ID NO: 661 - protein, 9 aa, Homo sapiens
ATSAVLALL

SEQ ID NO: 662 - protein, 9 aa, Homo sapiens
TGWAGGFFV

SEQ ID NO: 663 - protein, 9 aa, Homo sapiens
VLALLVMCI

SEQ ID NO: 664 - protein, 9 aa, Homo sapiens
ALLSCLLLT

SEQ ID NO: 665 - protein, 9 aa, Homo sapiens
CVAATLFWL

SEQ ID NO: 666 - protein, 9 aa, Homo sapiens
EMYSEIPEI

SEQ ID NO: 667 - protein, 9 aa, Homo sapiens
KMASTLVVA

SEQ ID NO: 668 - protein, 9 aa, Homo sapiens
SIFDKIYST

SEQ ID NO: 669 - protein, 9 aa, Homo sapiens
TLFWLLLTL

SEQ ID NO: 670 - protein, 9 aa, Homo sapiens
VLLWEIFSL

SEQ ID NO: 671 - protein, 9 aa, Homo sapiens
WLKDGLPAT

SEQ ID NO: 672 - protein, 9 aa, Homo sapiens
ILLDISFPG

SEQ ID NO: 673 - protein, 9 aa, Homo sapiens
LLDISFPGL

SEQ ID NO: 674 - protein, 9 aa, Homo sapiens
LMDLSTTPL

SEQ ID NO: 675 - protein, 9 aa, Homo sapiens
RVSSYLVPI

SEQ ID NO: 676 - protein, 9 aa, Homo sapiens
SLSKILLDI

SEQ ID NO: 677 - protein, 9 aa, Homo sapiens
SQLSYSQEV

SEQ ID NO: 678 - protein, 9 aa, Homo sapiens
WAAELPFPA

SEQ ID NO: 679 - protein, 9 aa, Homo sapiens
LLNESETKV

SEQ ID NO: 680 - protein, 9 aa, Homo sapiens
RLVELLKDL

SEQ ID NO: 681 - protein, 9 aa, Homo sapiens
GLASTTPEA

SEQ ID NO: 682 - protein, 9 aa, Homo sapiens
RMAREVAAL

SEQ ID NO: 683 - protein, 9 aa, Homo sapiens
FLLSLAFYG

SEQ ID NO: 684 - protein, 9 aa, Homo sapiens
ILNPAQGFL

SEQ ID NO: 685 - protein, 9 aa, Homo sapiens
MAWGLATLL

SEQ ID NO: 686 - protein, 9 aa, Homo sapiens
RLALGLLQL

SEQ ID NO: 687 - protein, 9 aa, Homo sapiens
RLLLAGAEV

SEQ ID NO: 688 - protein, 9 aa, Homo sapiens
CLYTFLIST

SEQ ID NO: 689 - protein, 9 aa, Homo sapiens
FLISTTFGC

SEQ ID NO: 690 - protein, 9 aa, Homo sapiens
VLLDTNYNL

SEQ ID NO: 691 - protein, 9 aa, Homo sapiens
WLPFGFILI

SEQ ID NO: 692 - protein, 10 aa, Homo sapiens
WLPFGFILIL

SEQ ID NO: 693 - protein, 9 aa, Homo sapiens
ALYLLPLLA

SEQ ID NO: 694 - protein, 9 aa, Homo sapiens
FALYNLLAL

SEQ ID NO: 695 - protein, 9 aa, Homo sapiens
QLFLVLQAL

SEQ ID NO: 696 - protein, 9 aa, Homo sapiens
RLVAAVVLL

SEQ ID NO: 697 - protein, 9 aa, Homo sapiens
VLAERAGAV

SEQ ID NO: 698 - protein, 9 aa, Homo sapiens
WLVPLFFAA

SEQ ID NO: 699 - protein, 9 aa, Homo sapiens
YLLPLLATC

SEQ ID NO: 700 - protein, 9 aa, Homo sapiens
GLSDAVEAL

SEQ ID NO: 701 - protein, 9 aa, Homo sapiens
MLREAAMGI

SEQ ID NO: 702 - protein, 9 aa, Homo sapiens
ALIPAPELV

SEQ ID NO: 703 - protein, 9 aa, Homo sapiens
NLLHGLNLL

SEQ ID NO: 704 - protein, 9 aa, Homo sapiens
YVSSLPQPL

SEQ ID NO: 705 - protein, 9 aa, Homo sapiens
YLILGVAGS

SEQ ID NO: 706 - protein, 9 aa, Homo sapiens
NMDCIIAEI

SEQ ID NO: 707 - protein, 9 aa, Homo sapiens
AVLGIFIIV

SEQ ID NO: 708 - protein, 9 aa, Homo sapiens
KLAVLGIFI

SEQ ID NO: 709 - protein, 9 aa, Homo sapiens
AIAAIVIGI

SEQ ID NO: 710 - protein, 9 aa, Homo sapiens
ALACSLAAC

SEQ ID NO: 711 - protein, 9 aa, Homo sapiens
IVIGIVALA

SEQ ID NO: 712 - protein, 9 aa, Homo sapiens
RIVAVPTPL

SEQ ID NO: 713 - protein, 9 aa, Homo sapiens
SLKELSPGI

SEQ ID NO: 714 - protein, 9 aa, Homo sapiens
KVADLVGFL

SEQ ID NO: 715 - protein, 9 aa, Homo sapiens
GMLSDVQSM

SEQ ID NO: 716 - protein, 9 aa, Homo sapiens
ILILILSIV

SEQ ID NO: 717 - protein, 9 aa, Homo sapiens
AMDAIFGSL

SEQ ID NO: 718 - protein, 9 aa, Homo sapiens
GLITKAEML

SEQ ID NO: 719 - protein, 9 aa, Homo sapiens
GTLEELPAA

SEQ ID NO: 720 - protein, 9 aa, Homo sapiens
KVLEYIANA

SEQ ID NO: 721 - protein, 9 aa, Homo sapiens
QLVFGIEVV

SEQ ID NO: 722 - protein, 9 aa, Homo sapiens
AVSSSSPLV

SEQ ID NO: 723 - protein, 9 aa, Homo sapiens
KVDELAHFL

SEQ ID NO: 724 - protein, 9 aa, Homo sapiens
KVLEHVVRV

SEQ ID NO: 725 - protein, 9 aa, Homo sapiens
VILGVLLLI

SEQ ID NO: 726 - protein, 9 aa, Homo sapiens
MTAAGVPQL

SEQ ID NO: 727 - protein, 9 aa, Homo sapiens
SVSDILSPL

SEQ ID NO: 728 - protein, 9 aa, Homo sapiens
ALLAASVAL

SEQ ID NO: 729 - protein, 9 aa, Homo sapiens
LLAASVALA

SEQ ID NO: 730 - protein, 9 aa, Homo sapiens
QLLRKVAEL

SEQ ID NO: 731 - protein, 9 aa, Homo sapiens
TLPELYAFT

SEQ ID NO: 732 - protein, 9 aa, Homo sapiens
YLYGKIKKT

SEQ ID NO: 733 - protein, 9 aa, Homo sapiens
QVLGLAAYL

SEQ ID NO: 734 - protein, 9 aa, Homo sapiens
GLDEVKSSL

SEQ ID NO: 735 - protein, 9 aa, Homo sapiens
FVLLSLSGA

SEQ ID NO: 736 - protein, 9 aa, Homo sapiens
SLFLFSVLL

SEQ ID NO: 737 - protein, 9 aa, Homo sapiens
SLTVYLVVA

SEQ ID NO: 738 - protein, 9 aa, Homo sapiens
VLLFVAVRL

SEQ ID NO: 739 - protein, 9 aa, Homo sapiens
VSSLFLFSV

SEQ ID NO: 740 - protein, 9 aa, Homo sapiens
SIAGFVASI

SEQ ID NO: 741 - protein, 9 aa, Homo sapiens
ILLVLMAVV

SEQ ID NO: 742 - protein, 9 aa, Homo sapiens
LIVGILLVL

SEQ ID NO: 743 - protein, 9 aa, Homo sapiens
LMAVVLASL

SEQ ID NO: 744 - protein, 9 aa, Homo sapiens
PLLDGTATL

SEQ ID NO: 745 - protein, 9 aa, Homo sapiens
SLADTNSLA

SEQ ID NO: 746 - protein, 9 aa, Homo sapiens
VLQAAIPLT

SEQ ID NO: 747 - protein, 9 aa, Homo sapiens
AVLDGLDVL

SEQ ID NO: 748 - protein, 9 aa, Homo sapiens
QLLALLPSL

SEQ ID NO: 749 - protein, 9 aa, Homo sapiens
RLRELLCEL

SEQ ID NO: 750 - protein, 9 aa, Homo sapiens
VLYPVPLES

SEQ ID NO: 751 - protein, 9 aa, Homo sapiens
AVFLLSYAV

SEQ ID NO: 752 - protein, 9 aa, Homo sapiens
FVLSLLLIL

SEQ ID NO: 753 - protein, 9 aa, Homo sapiens
IIFVLSLLL

SEQ ID NO: 754 - protein, 9 aa, Homo sapiens
LILEKQAAV

SEQ ID NO: 755 - protein, 9 aa, Homo sapiens
LISELKLAV

SEQ ID NO: 756 - protein, 9 aa, Homo sapiens
RAIEHVLQV

SEQ ID NO: 757 - protein, 9 aa, Homo sapiens
SSFDRLIPL

SEQ ID NO: 758 - protein, 9 aa, Homo sapiens
TLKEQFQFV

SEQ ID NO: 759 - protein, 9 aa, Homo sapiens
AILDSAFLL

SEQ ID NO: 760 - protein, 9 aa, Homo sapiens
AISLVFSLV

SEQ ID NO: 761 - protein, 9 aa, Homo sapiens
ALQILPYTL

SEQ ID NO: 762 - protein, 9 aa, Homo sapiens
ALTGFTFSA

SEQ ID NO: 763 - protein, 9 aa, Homo sapiens
AQLLLVNLL

SEQ ID NO: 764 - protein, 9 aa, Homo sapiens
CLFGLLTLI

SEQ ID NO: 765 - protein, 9 aa, Homo sapiens
GILLSLFLI

SEQ ID NO: 766 - protein, 9 aa, Homo sapiens
GLLPPPPAL

SEQ ID NO: 767 - protein, 9 aa, Homo sapiens
GLLTLIFLT

SEQ ID NO: 768 - protein, 9 aa, Homo sapiens
GLVAIYFAT

SEQ ID NO: 769 - protein, 9 aa, Homo sapiens
NLGALLPRL

SEQ ID NO: 770 - protein, 9 aa, Homo sapiens
SVAAFPVAA

SEQ ID NO: 771 - protein, 9 aa, Homo sapiens
FLLSLFCVT

SEQ ID NO: 772 - protein, 9 aa, Homo sapiens
FSLGVGFGV

SEQ ID NO: 773 - protein, 9 aa, Homo sapiens
GLIDEFQLL

SEQ ID NO: 774 - protein, 9 aa, Homo sapiens
GMESVITGL

SEQ ID NO: 775 - protein, 9 aa, Homo sapiens
ILFGVLIEA

SEQ ID NO: 776 - protein, 9 aa, Homo sapiens
KIDFLLSVI

SEQ ID NO: 777 - protein, 9 aa, Homo sapiens
LLFMVIAGM

SEQ ID NO: 778 - protein, 9 aa, Homo sapiens
LVPYLLFMV

SEQ ID NO: 779 - protein, 9 aa, Homo sapiens
QLTACLVLV

SEQ ID NO: 780 - protein, 9 aa, Homo sapiens
MISEKMVKL

SEQ ID NO: 781 - protein, 9 aa, Homo sapiens
LMFDLSLNF

SEQ ID NO: 782 - protein, 9 aa, Homo sapiens
ALPAVMAGL

SEQ ID NO: 783 - protein, 9 aa, Homo sapiens
GLAEPQAAA

SEQ ID NO: 784 - protein, 9 aa, Homo sapiens
GIFLLSALA

SEQ ID NO: 785 - protein, 9 aa, Homo sapiens
ASLTFLYTL

SEQ ID NO: 786 - protein, 9 aa, Homo sapiens
AVLHAIYSL

SEQ ID NO: 787 - protein, 9 aa, Homo sapiens
FFFAVLHAI

SEQ ID NO: 788 - protein, 9 aa, Homo sapiens
GVIAAIVQL

SEQ ID NO: 789 - protein, 9 aa, Homo sapiens
KIAAIIASL

SEQ ID NO: 790 - protein, 9 aa, Homo sapiens
LIFKSILFL

SEQ ID NO: 791 - protein, 9 aa, Homo sapiens
LLLGTIHAL

SEQ ID NO: 792 - protein, 9 aa, Homo sapiens
LLSFFFAVL

SEQ ID NO: 793 - protein, 9 aa, Homo sapiens
MIAVFLPIV

SEQ ID NO: 794 - protein, 9 aa, Homo sapiens
SLLLGTIHA

SEQ ID NO: 795 - protein, 9 aa, Homo sapiens
SLSLIVAVI

SEQ ID NO: 796 - protein, 9 aa, Homo sapiens
IISPNLFYA

SEQ ID NO: 797 - protein, 9 aa, Homo sapiens
LLDHVLIEM

SEQ ID NO: 798 - protein, 9 aa, Homo sapiens
VLIDEHLVL

SEQ ID NO: 799 - protein, 9 aa, Homo sapiens
YSSEVLEYM

SEQ ID NO: 800 - protein, 9 aa, Homo sapiens
ILLRPDTYI

SEQ ID NO: 801 - protein, 9 aa, Homo sapiens
LMMTIINLA

SEQ ID NO: 802 - protein, 9 aa, Homo sapiens
QLAGSVAEM

SEQ ID NO: 803 - protein, 9 aa, Homo sapiens
SLMMTIINL

SEQ ID NO: 804 - protein, 9 aa, Homo sapiens
TMLSSLARL

SEQ ID NO: 805 - protein, 9 aa, Homo sapiens
YIFTMLSSL

SEQ ID NO: 806 - protein, 9 aa, Homo sapiens
DLAGVIIEL

SEQ ID NO: 807 - protein, 9 aa, Homo sapiens
FGLFGVFLV

SEQ ID NO: 808 - protein, 9 aa, Homo sapiens
GLFGVFLVL

SEQ ID NO: 809 - protein, 9 aa, Homo sapiens
ILDTAIIVI

SEQ ID NO: 810 - protein, 9 aa, Homo sapiens
IVSSFAFGL

SEQ ID NO: 811 - protein, 9 aa, Homo sapiens
RLLRLIILL

SEQ ID NO: 812 - protein, 9 aa, Homo sapiens
SLAIALFFL

SEQ ID NO: 813 - protein, 9 aa, Homo sapiens
YFWLHTSFI

SEQ ID NO: 814 - protein, 9 aa, Homo sapiens
AMFGYTVGT

SEQ ID NO: 815 - protein, 9 aa, Homo sapiens
FIAGIVFRL

SEQ ID NO: 816 - protein, 9 aa, Homo sapiens
FLLLFAYVL

SEQ ID NO: 817 - protein, 9 aa, Homo sapiens
LLFAYVLLM

SEQ ID NO: 818 - protein, 9 aa, Homo sapiens
LLLFAYVLL

SEQ ID NO: 819 - protein, 9 aa, Homo sapiens
LVLYSLVFV

SEQ ID NO: 820 - protein, 9 aa, Homo sapiens
NILLVNLLV

SEQ ID NO: 821 - protein, 9 aa, Homo sapiens
QIADVIASL

SEQ ID NO: 822 - protein, 9 aa, Homo sapiens
VLYSLVFVL

SEQ ID NO: 823 - protein, 9 aa, Homo sapiens
YLVKINTKA

SEQ ID NO: 824 - protein, 9 aa, Homo sapiens
FLDSLGFST

SEQ ID NO: 825 - protein, 9 aa, Homo sapiens
SLRDEFPLL

SEQ ID NO: 826 - protein, 9 aa, Homo sapiens
VLEELLWFI

SEQ ID NO: 827 - protein, 9 aa, Homo sapiens
ALLAGLVSL

SEQ ID NO: 828 - protein, 9 aa, Homo sapiens
AMVGAVLTA

SEQ ID NO: 829 - protein, 9 aa, Homo sapiens
ISSDYVIPI

SEQ ID NO: 830 - protein, 9 aa, Homo sapiens
LLAGLVSLL

SEQ ID NO: 831 - protein, 9 aa, Homo sapiens
LLSPASFFS

SEQ ID NO: 832 - protein, 9 aa, Homo sapiens
MVGAVLTAL

SEQ ID NO: 833 - protein, 9 aa, Homo sapiens
VLTALLAGL

SEQ ID NO: 834 - protein, 9 aa, Homo sapiens
ALTESLLVA

SEQ ID NO: 835 - protein, 9 aa, Homo sapiens
LLALLSPGA

SEQ ID NO: 836 - protein, 9 aa, Homo sapiens
LVLGFIIAL

SEQ ID NO: 837 - protein, 9 aa, Homo sapiens
SLSGLLSPA

SEQ ID NO: 838 - protein, 9 aa, Homo sapiens
TLPLILILL

SEQ ID NO: 839 - protein, 9 aa, Homo sapiens
VLGFIIALA

SEQ ID NO: 840 - protein, 9 aa, Homo sapiens
VVITVLLSV

SEQ ID NO: 841 - protein, 9 aa, Homo sapiens
AQIGDSVML

SEQ ID NO: 842 - protein, 9 aa, Homo sapiens
FASSLIIPA

SEQ ID NO: 843 - protein, 9 aa, Homo sapiens
KSIDGAYTI

SEQ ID NO: 844 - protein, 9 aa, Homo sapiens
SILEEGSSV

SEQ ID NO: 845 - protein, 9 aa, Homo sapiens
LLFGFTLVS

SEQ ID NO: 846 - protein, 9 aa, Homo sapiens
LLLFGFTLV

SEQ ID NO: 847 - protein, 9 aa, Homo sapiens
RLGPLAAAL

SEQ ID NO: 848 - protein, 9 aa, Homo sapiens
DLNALLPAV

SEQ ID NO: 849 - protein, 9 aa, Homo sapiens
ILIPQVAYT

SEQ ID NO: 850 - protein, 9 aa, Homo sapiens
NLSDIQNVL

SEQ ID NO: 851 - protein, 9 aa, Homo sapiens
VQAVVLPTV

SEQ ID NO: 852 - protein, 9 aa, Homo sapiens
LVLEQFLTI

SEQ ID NO: 853 - protein, 9 aa, Homo sapiens
RISGYISEA

SEQ ID NO: 854 - protein, 9 aa, Homo sapiens
AMTDISSLA

SEQ ID NO: 855 - protein, 9 aa, Homo sapiens
VLLSNFYYG

SEQ ID NO: 856 - protein, 20 aa, synthetic construct
  REGION 1..20: note = peptide
MAKTIAYDEEARRGLERGLN

SEQ ID NO: 857 - protein, 9 aa, Homo sapiens
QLWQFLLEL

SEQ ID NO: 858 - protein, 9 aa, Homo sapiens
LVLGTLEEV

SEQ ID NO: 859 - protein, 15 aa, synthetic construct
  REGION 1..15: note = peptide
KSVWSKLQSIGIRQH

SEQ ID NO: 860 - protein, 13 aa, synthetic construct
  REGION 1..13: note = peptide
TPPAYRPPNAPIL

SEQ ID NO: 861 - protein, 9 aa, synthetic construct
  REGION 1..9: note = peptide
WLLDISFPL

SEQ ID NO: 862 - protein, 9 aa, synthetic construct
  REGION 1..9: note = peptide
HLLDISFPA

SEQ ID NO: 863 - protein, 9 aa, synthetic construct
  REGION 1..9: note = peptide
ELLDISFPA

SEQ ID NO: 864 - protein, 9 aa, synthetic construct
  REGION 1..9: note = peptide
VLLDISFEL

SEQ ID NO: 865 - protein, 9 aa, synthetic construct
  REGION 1..9: note = peptide
VLLDISFKV

SEQ ID NO: 866 - protein, 9 aa, synthetic construct
  REGION 1..9: note = peptide
IMLDISFLL

SEQ ID NO: 867 - protein, 9 aa, synthetic construct
  REGION 1..9: note = peptide
LLDISFPSL

SEQ ID NO: 868 - protein, 9 aa, synthetic construct
  REGION 1..9: note = peptide
LMDLSTTNV

SEQ ID NO: 869 - protein, 9 aa, synthetic construct
  REGION 1..9: note = peptide
MLSSYLVPI

SEQ ID NO: 870 - protein, 9 aa, synthetic construct
  REGION 1..9: note = peptide
LLSSYLVPI

SEQ ID NO: 871 - protein, 9 aa, synthetic construct
  REGION 1..9: note = peptide
FVSSYLVPT

SEQ ID NO: 872 - protein, 9 aa, synthetic construct
  REGION 1..9: note = peptide
SLSLHDMFL

SEQ ID NO: 873 - protein, 9 aa, synthetic construct
  REGION 1..9: note = peptide
KLKPLLPWI

SEQ ID NO: 874 - protein, 9 aa, synthetic construct
  REGION 1..9: note = peptide
KLKPLLPFL

SEQ ID NO: 875 - protein, 9 aa, synthetic construct
  REGION 1..9: note = peptide
KVVPIQFPV

SEQ ID NO: 876 - protein, 9 aa, synthetic construct
  REGION 1..9: note = peptide
KIVPIQFPI

SEQ ID NO: 877 - protein, 9 aa, synthetic construct
  REGION 1..9: note = peptide
YQAMIQFLI

SEQ ID NO: 878 - protein, 10 aa, synthetic construct
  REGION 1..10: note = peptide
FMPFGFILPI

SEQ ID NO: 879 - protein, 10 aa, synthetic construct
  REGION 1..10: note = peptide
FMPFGFILGV

SEQ ID NO: 880 - protein, 10 aa, synthetic construct
  REGION 1..10: note = peptide
FLISTTFTIN

SEQ ID NO: 881 - protein, 10 aa, synthetic construct
  REGION 1..10: note = peptide
FMISTTFMRL

SEQ ID NO: 882 - protein, 10 aa, synthetic construct
  REGION 1..10: note = peptide
QMISTTFGNV

SEQ ID NO: 883 - protein, 10 aa, synthetic construct
  REGION 1..10: note = peptide
WLYLQWQPSV

SEQ ID NO: 884 - protein, 10 aa, synthetic construct
  REGION 1..10: note = peptide
FVLLDTNYEI

SEQ ID NO: 885 - protein, 10 aa, synthetic construct
  REGION 1..10: note = peptide
FILLDTNYEI

SEQ ID NO: 886 - protein, 10 aa, synthetic construct
  REGION 1..10: note = peptide
YELQNIVLPI

SEQ ID NO: 887 - protein, 10 aa, synthetic construct
  REGION 1..10: note = peptide
FMLQNIVKNL

SEQ ID NO: 888 - protein, 9 aa, Homo sapiens
NLSLHDMFV

SEQ ID NO: 889 - protein, 9 aa, Homo sapiens
KMKPLLPRV

SEQ ID NO: 890 - protein, 9 aa, Homo sapiens
YLVPIQFPV

SEQ ID NO: 891 - protein, 9 aa, Homo sapiens
YMAMIQFAI

SEQ ID NO: 892 - protein, 10 aa, Homo sapiens
FLISTTFGCT

SEQ ID NO: 893 - protein, 10 aa, Homo sapiens
YLYLQWQPPL

SEQ ID NO: 894 - protein, 10 aa, Homo sapiens
GVLLDTNYNL

SEQ ID NO: 895 - protein, 10 aa, Homo sapiens
FQLQNIVKPL

SEQ ID NO: 896 - protein, 9 aa, synthetic construct
  REGION 1..9: note = comparative peptide
ALPFGFILV

SEQ ID NO: 897 - protein, 9 aa, synthetic construct
  REGION 1..9: note = comparative peptide
ILPFGFILA

SEQ ID NO: 898 - protein, 9 aa, synthetic construct
  REGION 1..9: note = comparative peptide
FLPFGFILM

SEQ ID NO: 899 - protein, 9 aa, synthetic construct
  REGION 1..9: note = comparative peptide
LMLGEFLKL